European Patent Application EP 4 715 058 A1, published March 25, 2026. Title: 一种Rett综合症的基因治疗. Applicant: 上海金珂博生物技术有限公司. Application WO. The sequence listing filed with the application follows.

SEQUENCE LISTING (75 sequences)

SEQ ID NO: 1 - protein, 498 aa, synthetic construct [sequence omitted]

SEQ ID NO: 2 - DNA, 61 bp, synthetic construct
  source 1..61: mol_type = other DNA
acaagaataaaggcagctgttgtctcttctccttatgggtagggctctgacaaagcttccc

SEQ ID NO: 3 - DNA, 200 bp, synthetic construct
  source 1..200: mol_type = other DNA
atatcaccaggactgttaatatatttaaaaacaaaaggcaatttattaaggaaatttgtaccatttcagtaaacctgtctgaatgtacctgtatacgtttcaaaaacaccccccccccactgaatccctgtaacctatttattatataaagagtttgccttataaatttacataaaaatgtccgtttgtgtcttttgttg

SEQ ID NO: 4 - DNA, 22 bp, synthetic construct
  source 1..22: mol_type = other DNA
ctcccttctttcctcccgtcta

SEQ ID NO: 5 - DNA, 22 bp, synthetic construct
  source 1..22: mol_type = other DNA
atgcccttttaacattgcacta

SEQ ID NO: 6 - DNA, 22 bp, synthetic construct
  source 1..22: mol_type = other DNA
cgaccatggctgtagactgtta

SEQ ID NO: 7 - DNA, 22 bp, synthetic construct
  source 1..22: mol_type = other DNA
ttggcattcaccgcgtgcctta

SEQ ID NO: 8 - DNA, 49 bp, synthetic construct
  source 1..49: mol_type = other DNA
aataaaagatctttattttcattagatctgtgtgttggttttttgtgtg

SEQ ID NO: 9 - DNA, 22 bp, synthetic construct
  source 1..22: mol_type = other DNA
agtgaattctaccagtgccata

SEQ ID NO: 10 - DNA, 22 bp, synthetic construct
  source 1..22: mol_type = other DNA
caaacaccattgtcacactcca

SEQ ID NO: 11 - DNA, 22 bp, synthetic construct
  source 1..22: mol_type = other DNA
gtacctgtatacgtttcaaaaa

SEQ ID NO: 12 - DNA, 20 bp, synthetic construct
  source 1..20: mol_type = other DNA
caccccccccccactgaatc

SEQ ID NO: 13 - DNA, 18 bp, synthetic construct
  source 1..18: mol_type = other DNA
cctgtaacctatttatta

SEQ ID NO: 14 - DNA, 549 bp, synthetic construct
  source 1..549: mol_type = other DNA
tggaacaacgccaggctcctcaacaggcaactttgctacttctacagaaaatgataataaagaaatgctggtgaagtcaaatgcttatcacaatggtgaactactcagcagggaggctctaataggcgccaagagcctagacttccttaagcgccagagtccacaagggcccagttaatcctcaacattcaaatgctgcccacaaaaccagcccctctgtgccctagccgcctcttttttccaagtgacagtagaactccaccaatccgcagctgaatggggtccgcctcttttccctgcctaaacagacaggaactcctgccaattgagggcgtcaccgctaaggctccgccccagcctgggctccacaaccaatgaagggtaatctcgacaaagagcaaggggtggggcgcgggcgcgcaggtgcagcagcacacaggctggtcgggagggcggggcgcgacgtctgccgtgcggggtcccggcatcggttgcgcgcgcgctccctcctctcggagagagggctgtggtaaaacccgtccggaaaac

SEQ ID NO: 15 - DNA, 426 bp, synthetic construct
  source 1..426: mol_type = other DNA
ataggcgccaagagcctagacttccttaagcgccagagtccacaagggcccagttaatcctcaacattcaaatgctgcccacaaaaccagcccctctgtgccctagccgcctcttttttccaagtgacagtagaactccaccaatccgcagctgaatggggtccgcctcttttccctgcctaaacagacaggaactcctgccaattgagggcgtcaccgctaaggctccgccccagcctgggctccacaaccaatgaagggtaatctcgacaaagagcaaggggtggggcgcgggcgcgcaggtgcagcagcacacaggctggtcgggagggcggggcgcgacgtctgccgtgcggggtcccggcatcggttgcgcgcgcgctccctcctctcggagagagggctgtggtaaaacccgtccggaaa

SEQ ID NO: 16 - DNA, 322 bp, synthetic construct
  source 1..322: mol_type = other DNA
agccgcctcttttttccaagtgacagtagaactccaccaatccgcagctgaatggggtccgcctcttttccctgcctaaacagacaggaactcctgccaattgagggcgtcaccgctaaggctccgccccagcctgggctccacaaccaatgaagggtaatctcgacaaagagcaaggggtggggcgcgggcgcgcaggtgcagcagcacacaggctggtcgggagggcggggcgcgacgtctgccgtgcggggtcccggcatcggttgcgcgcgcgctccctcctctcggagagagggctgtggtaaaacccgtccggaaa

SEQ ID NO: 17 - DNA, 223 bp, synthetic construct
  source 1..223: mol_type = other DNA
attgagggcgtcaccgctaaggctccgccccagcctgggctccacaaccaatgaagggtaatctcgacaaagagcaaggggtggggcgcgggcgcgcaggtgcagcagcacacaggctggtcgggagggcggggcgcgacgtctgccgtgcggggtcccggcatcggttgcgcgcgcgctccctcctctcggagagagggctgtggtaaaacccgtccggaaa

SEQ ID NO: 18 - DNA, 1777 bp, synthetic construct
  source 1..1777: mol_type = other DNA
atggccgccgccgccgccgccgcgccgagcggaggaggaggaggaggcgaggaggagagactggaagaaaagtcagaagaccaggacctccagggcctcaaggacaaacccctcaagtttaaaaaggtgaagaaagataagaaagaagagaaagagggcaagcatgagcccgtgcagccatcagcccaccactctgctgagcccgcagaggcaggcaaagcagagacatcagaagggtcaggctccgccccggctgtgccggaagcttctgcctcccccaaacagcggcgctccatcatccgtgaccggggacccatgtatgatgaccccaccctgcctgaaggctggacacggaagcttaagcaaaggaaatctggccgctctgctgggaagtatgatgtgtatttgatcaatccccagggaaaagcctttcgctctaaagtggagttgattgcgtacttcgaaaaggtaggcgacacatccctggaccctaatgattttgacttcacggtaactgggagagggagcccctcccggcgagagcagaaaccacctaagaagcccaaatctcccaaagctccaggaactggcagaggccggggacgccccaaagggagcggcaccacgagacccaaggcggccacgtcagagggtgtgcaggtgaaaagggtcctggagaaaagtcctgggaagctccttgtcaagatgccttttcaaacttcgccagggggcaaggctgaggggggtggggccaccacatccacccaggtcatggtgatcaaacgccccggcaggaagcgaaaagctgaggccgaccctcaggccattcccaagaaacggggccgaaagccggggagtgtggtggcagccgctgccgccgaggccaaaaagaaagccgtgaaggagtcttctatccgatctgtgcaggagaccgtactccccatcaagaagcgcaagacccgggagacggtcagcatcgaggtcaaggaagtggtgaagcccctgctggtgtccaccctcggtgagaagagcgggaaaggactgaagacctgtaagagccctgggcggaaaagcaaggagagcagccccaaggggcgcagcagcagcgcctcctcaccccccaagaaggagcaccaccaccatcaccaccactcagagtccccaaaggcccccgtgccactgctcccacccctgcccccacctccacctgagcccgagagctccgaggaccccaccagcccccctgagccccaggacttgagcagcagcgtctgcaaagaggagaagatgcccagaggaggctcactggagagcgacggctgccccaaggagccagctaagactcagcccgcggttgccaccgccgccacggccgcagaaaagtacaaacaccgaggggagggagagcgcaaagacattgtttcatcctccatgccaaggccaaacagagaggagcctgtggacagccggacgcccgtgaccgagagagttagcgggagctccggcagttctggagaacaaaaactcatctcagaagaggatctgtgaacaagaataaaggcagctgttgtctcttctccttatgggtagggctctgacaaagcttcccatatcaccaggactgttaatatatttaaaaacaaaaggcaatttattaaggaaatttgtaccatttcagtaaacctgtctgaaccggagagaccgagagagggtctcagttttataaagagtttgccttataaatttacataaaaatgtccgtttgtgtcttttgttg

SEQ ID NO: 19 - DNA, 1430 bp, synthetic construct
  source 1..1430: mol_type = other DNA
ataggcgccaagagcctagacttccttaagcgccagagtccacaagggcccagttaatcctcaacattcaaatgctgcccacaaaaccagcccctctgtgccctagccgcctcttttttccaagtgacagtagaactccaccaatccgcagctgaatggggtccgcctcttttccctgcctaaacagacaggaactcctgccaattgagggcgtcaccgctaaggctccgccccagcctgggctccacaaccaatgaagggtaatctcgacaaagagcaaggggtggggcgcgggcgcgcaggtgcagcagcacacaggctggtcgggagggcggggcgcgacgtctgccgtgcggggtcccggcatcggttgcgcgcgcgctccctcctctcggagagagggctgtggtaaaacccgtccggaaaccatggccgccgccgccgccgccgcgccgagcggaggaggaggaggaggcgaggaggagagactggaagaaaagccggctgtgccggaagcttctgcctcccccaaacagcggcgctccatcatccgtgaccggggacccatgtatgatgaccccaccctgcctgaaggctggacacggaagcttaagcaaaggaaatctggccgctctgctgggaagtatgatgtgtatttgatcaatccccagggaaaagcctttcgctctaaagtggagttgattgcgtacttcgaaaaggtaggcgacacatccctggaccctaatgattttgacttcacggtaactgggagagggagcccctcccggcgagagcagaaaccacctggatccagtggcagctctgggcccaagaaaaagcggaaggtgccggggagtgtggtggcagccgctgccgccgaggccaaaaagaaagccgtgaaggagtcttctatccgatctgtgcaggagaccgtactccccatcaagaagcgcaagacccgggagacggtcgggagctccggcagttctggagaacaaaaactcatctcagaagaggatctggtcgactagagctcgctgatcagcctcacaagaataaaggcagctgttgtctcttcagaagtagctttgcacttttctaaactaggaatatcaccaggactgttactcaatgtgtggtcgacctgttctagcccccaaagagttttctgtgcttgcttttgaaacttgaagtcttgaaaaccaaagacatagatgtgaaaattttaggcagtgtaagctgatagcacaagttctggcgactcacaattatgctgtgaattttacaaaaagaagcagtaatctacctcagccgataacgaaagcactgatatatttaaaaacaaaaggtgtaacctatttattatataaagagtttgccttataaatttacataaaaatgtccgtttgtgtcttttgttgtaaaaatca

SEQ ID NO: 20 - DNA, 2258 bp, synthetic construct
  source 1..2258: mol_type = other DNA
ctgcgcgctcgctcgctcactgaggccgcccgggcaaagcccgggcgtcgggcgacctttggtcgcccggcctcagtgagcgagcgagcgcgcagagagggagtggagtacttggaacaacgccaggctcctcaacaggcaactttgctacttctacagaaaatgataataaagaaatgctggtgaagtcaaatgcttatcacaatggtgaactactcagcagggaggctctaataggcgccaagagcctagacttccttaagcgccagagtccacaagggcccagttaatcctcaacattcaaatgctgcccacaaaaccagcccctctgtgccctagccgcctcttttttccaagtgacagtagaactccaccaatccgcagctgaatggggtccgcctcttttccctgcctaaacagacaggaactcctgccaattgagggcgtcaccgctaaggctccgccccagcctgggctccacaaccaatgaagggtaatctcgacaaagagcaaggggtggggcgcgggcgcgcaggtgcagcagcacacaggctggtcgggagggcggggcgcgacgtctgccgtgcggggtcccggcatcggttgcgcgcgcgctccctcctctcggagagagggctgtggtaaaacccgtccggaaaacatggccgccgccgccgccgccgcgccgagcggaggaggaggaggaggcgaggaggagagactggaagaaaagtcagaagaccaggacctccagggcctcaaggacaaacccctcaagtttaaaaaggtgaagaaagataagaaagaagagaaagagggcaagcatgagcccgtgcagccatcagcccaccactctgctgagcccgcagaggcaggcaaagcagagacatcagaagggtcaggctccgccccggctgtgccggaagcttctgcctcccccaaacagcggcgctccatcatccgtgaccggggacccatgtatgatgaccccaccctgcctgaaggctggacacggaagcttaagcaaaggaaatctggccgctctgctgggaagtatgatgtgtatttgatcaatccccagggaaaagcctttcgctctaaagtggagttgattgcgtacttcgaaaaggtaggcgacacatccctggaccctaatgattttgacttcacggtaactgggagagggagcccctcccggcgagagcagaaaccacctaagaagcccaaatctcccaaagctccaggaactggcagaggccggggacgccccaaagggagcggcaccacgagacccaaggcggccacgtcagagggtgtgcaggtgaaaagggtcctggagaaaagtcctgggaagctccttgtcaagatgccttttcaaacttcgccagggggcaaggctgaggggggtggggccaccacatccacccaggtcatggtgatcaaacgccccggcaggaagcgaaaagctgaggccgaccctcaggccattcccaagaaacggggccgaaagccggggagtgtggtggcagccgctgccgccgaggccaaaaagaaagccgtgaaggagtcttctatccgatctgtgcaggagaccgtactccccatcaagaagcgcaagacccgggagacggtcagcatcgaggtcaaggaagtggtgaagcccctgctggtgtccaccctcggtgagaagagcgggaaaggactgaagacctgtaagagccctgggcggaaaagcaaggagagcagccccaaggggcgcagcagcagcgcctcctcaccccccaagaaggagcaccaccaccatcaccaccactcagagtccccaaaggcccccgtgccactgctcccacccctgcccccacctccacctgagcccgagagctccgaggaccccaccagcccccctgagccccaggacttgagcagcagcgtctgcaaagaggagaagatgcccagaggaggctcactggagagcgacggctgccccaaggagccagctaagactcagcccgcggttgccaccgccgccacggccgcagaaaagtacaaacaccgaggggagggagagcgcaaagacattgtttcatcctccatgccaaggccaaacagagaggagcctgtggacagccggacgcccgtgaccgagagagttagcgggagctccggcagttctggagaacaaaaactcatctcagaagaggatctgtgaaataaaagatctttattttcattagatctgtgtgttggttttttgtgtg

SEQ ID NO: 21 - DNA, 1541 bp, synthetic construct
  source 1..1541: mol_type = other DNA
ctgcgcgctcgctcgctcactgaggccgcccgggcaaagcccgggcgtcgggcgacctttggtcgcccggcctcagtgagcgagcgagcgcgcagagagggagtggagtactataggcgccaagagcctagacttccttaagcgccagagtccacaagggcccagttaatcctcaacattcaaatgctgcccacaaaaccagcccctctgtgccctagccgcctcttttttccaagtgacagtagaactccaccaatccgcagctgaatggggtccgcctcttttccctgcctaaacagacaggaactcctgccaattgagggcgtcaccgctaaggctccgccccagcctgggctccacaaccaatgaagggtaatctcgacaaagagcaaggggtggggcgcgggcgcgcaggtgcagcagcacacaggctggtcgggagggcggggcgcgacgtctgccgtgcggggtcccggcatcggttgcgcgcgcgctccctcctctcggagagagggctgtggtaaaacccgtccggaaaccatggccgccgccgccgccgccgcgccgagcggaggaggaggaggaggcgaggaggagagactggaagaaaagccggctgtgccggaagcttctgcctcccccaaacagcggcgctccatcatccgtgaccggggacccatgtatgatgaccccaccctgcctgaaggctggacacggaagcttaagcaaaggaaatctggccgctctgctgggaagtatgatgtgtatttgatcaatccccagggaaaagcctttcgctctaaagtggagttgattgcgtacttcgaaaaggtaggcgacacatccctggaccctaatgattttgacttcacggtaactgggagagggagcccctcccggcgagagcagaaaccacctggatccagtggcagctctgggcccaagaaaaagcggaaggtgccggggagtgtggtggcagccgctgccgccgaggccaaaaagaaagccgtgaaggagtcttctatccgatctgtgcaggagaccgtactccccatcaagaagcgcaagacccgggagacggtcgggagctccggcagttctggagaacaaaaactcatctcagaagaggatctggtcgactaggctcgctgatcagcctcacaagaataaaggcagctgttgtctcttcagaagtagctttgcacttttctaaactaggaatatcaccaggactgttactcaatgtgtggtcgacctgttctagcccccaaagagttttctgtgcttgcttttgaaacttgaagtcttgaaaaccaaagacatagatgtgaaaattttaggcagtgtaagctgatagcacaagttctggcgactcacaattatgctgtgaattttacaaaaagaagcagtaatctacctcagccgataacgaaagcactgatatatttaaaaacaaaaggtgtaacctatttattatataaagagtttgccttataaatttacataaaaatgtccgtttgtgtcttttgttgtaaaaatca

SEQ ID NO: 22 - DNA, 45 bp, synthetic construct
  source 1..45: mol_type = other DNA
gcagagagggagtggagtacttggaacaacgccaggctcctcaac

SEQ ID NO: 23 - DNA, 43 bp, synthetic construct
  source 1..43: mol_type = other DNA
gcggcggcggcggccatgttttccggacgggttttaccacagc

SEQ ID NO: 24 - DNA, 17 bp, synthetic construct
  source 1..17: mol_type = other DNA
atggccgccgccgccgc

SEQ ID NO: 25 - DNA, 33 bp, synthetic construct
  source 1..33: mol_type = other DNA
tcacagatcctcttctgagatgagtttttgttc

SEQ ID NO: 26 - DNA, 52 bp, synthetic construct
  source 1..52: mol_type = other DNA
tcagaagaggatctgtgaaataaaagatctttattttcattagatctgtgtg

SEQ ID NO: 27 - DNA, 46 bp, synthetic construct
  source 1..46: mol_type = other DNA
tcactaggggttcctagtactcacacaaaaaaccaacacacagatc

SEQ ID NO: 28 - DNA, 45 bp, synthetic construct
  source 1..45: mol_type = other DNA
gcagagagggagtggagtactataggcgccaagagcctagacttc

SEQ ID NO: 29 - DNA, 45 bp, synthetic construct
  source 1..45: mol_type = other DNA
gcagagagggagtggagtactagccgcctcttttttccaagtgac

SEQ ID NO: 30 - DNA, 42 bp, synthetic construct
  source 1..42: mol_type = other DNA
gcagagagggagtggagtactattgagggcgtcaccgctaag

SEQ ID NO: 31 - DNA, 43 bp, synthetic construct
  source 1..43: mol_type = other DNA
ggcggcggcggcggccatggtttccggacgggttttaccacag

SEQ ID NO: 32 - DNA, 46 bp, synthetic construct; identical to SEQ ID NO: 27
  source 1..46: mol_type = other DNA

SEQ ID NO: 33 - skipped

SEQ ID NO: 34 - DNA, 87 bp, synthetic construct
  source 1..87: mol_type = other DNA
attaaggaaatttgtaccagtgaattctaccagtgccatagtacctgtatacgtttcaaaaactcccttctttcctcccgtctacac

SEQ ID NO: 35 - DNA, 82 bp, synthetic construct
  source 1..82: mol_type = other DNA
taaggcaaactctttatatggagtgtgacaatggtgtttggattcagtggggggggggtgtagacgggaggaaagaagggag

SEQ ID NO: 36 - DNA, 109 bp, synthetic construct
  source 1..109: mol_type = other DNA
attaaggaaatttgtaccagtgaattctaccagtgccatagtacctgtatacgtttcaaaaactcccttctttcctcccgtctacaccccccccccactgaatccaaac

SEQ ID NO: 37 - DNA, 104 bp, synthetic construct
  source 1..104: mol_type = other DNA
taaggcaaactctttatataaggcacgcggtgaatgccaataataaataggttacaggtggagtgtgacaatggtgtttggattcagtggggggggggtgtaga

SEQ ID NO: 38 - DNA, 109 bp, synthetic construct; identical to SEQ ID NO: 36
  source 1..109: mol_type = other DNA

SEQ ID NO: 39 - DNA, 104 bp, synthetic construct
  source 1..104: mol_type = other DNA
taaggcaaactctttatatagtgcaatgttaaaagggcattaataaataggttacaggtggagtgtgacaatggtgtttggattcagtggggggggggtgtaga

SEQ ID NO: 40 - DNA, 109 bp, synthetic construct; identical to SEQ ID NO: 36
  source 1..109: mol_type = other DNA

SEQ ID NO: 41 - DNA, 104 bp, synthetic construct
  source 1..104: mol_type = other DNA
taaggcaaactctttatataacagtctacagccatggtcgtaataaataggttacaggtggagtgtgacaatggtgtttggattcagtggggggggggtgtaga

SEQ ID NO: 42 - DNA, 2205 bp, synthetic construct
  source 1..2205: mol_type = other DNA
ataggcgccaagagcctagacttccttaagcgccagagtccacaagggcccagttaatcctcaacattcaaatgctgcccacaaaaccagcccctctgtgccctagccgcctcttttttccaagtgacagtagaactccaccaatccgcagctgaatggggtccgcctcttttccctgcctaaacagacaggaactcctgccaattgagggcgtcaccgctaaggctccgccccagcctgggctccacaaccaatgaagggtaatctcgacaaagagcaaggggtggggcgcgggcgcgcaggtgcagcagcacacaggctggtcgggagggcggggcgcgacgtctgccgtgcggggtcccggcatcggttgcgcgcgcgctccctcctctcggagagagggctgtggtaaaacccgtccggaaaccatggccgccgccgccgccgccgcgccgagcggaggaggaggaggaggcgaggaggagagactggaagaaaagtcagaagaccaggacctccagggcctcaaggacaaacccctcaagtttaaaaaggtgaagaaagataagaaagaagagaaagagggcaagcatgagcccgtgcagccatcagcccaccactctgctgagcccgcagaggcaggcaaagcagagacatcagaagggtcaggctccgccccggctgtgccggaagcttctgcctcccccaaacagcggcgctccatcatccgtgaccggggacccatgtatgatgaccccaccctgcctgaaggctggacacggaagcttaagcaaaggaaatctggccgctctgctgggaagtatgatgtgtatttgatcaatccccagggaaaagcctttcgctctaaagtggagttgattgcgtacttcgaaaaggtaggcgacacatccctggaccctaatgattttgacttcacggtaactgggagagggagcccctcccggcgagagcagaaaccacctaagaagcccaaatctcccaaagctccaggaactggcagaggccggggacgccccaaagggagcggcaccacgagacccaaggcggccacgtcagagggtgtgcaggtgaaaagggtcctggagaaaagtcctgggaagctccttgtcaagatgccttttcaaacttcgccagggggcaaggctgaggggggtggggccaccacatccacccaggtcatggtgatcaaacgccccggcaggaagcgaaaagctgaggccgaccctcaggccattcccaagaaacggggccgaaagccggggagtgtggtggcagccgctgccgccgaggccaaaaagaaagccgtgaaggagtcttctatccgatctgtgcaggagaccgtactccccatcaagaagcgcaagacccgggagacggtcagcatcgaggtcaaggaagtggtgaagcccctgctggtgtccaccctcggtgagaagagcgggaaaggactgaagacctgtaagagccctgggcggaaaagcaaggagagcagccccaaggggcgcagcagcagcgcctcctcaccccccaagaaggagcaccaccaccatcaccaccactcagagtccccaaaggcccccgtgccactgctcccacccctgcccccacctccacctgagcccgagagctccgaggaccccaccagcccccctgagccccaggacttgagcagcagcgtctgcaaagaggagaagatgcccagaggaggctcactggagagcgacggctgccccaaggagccagctaagactcagcccgcggttgccaccgccgccacggccgcagaaaagtacaaacaccgaggggagggagagcgcaaagacattgtttcatcctccatgccaaggccaaacagagaggagcctgtggacagccggacgcccgtgaccgagagagttagcgggagctccggcagttctggagaacaaaaactcatctcagaagaggatctgtgaacaagaataaaggcagctgttgtctcttctccttatgggtagggctctgacaaagcttcccatatcaccaggactgttaatatatttaaaaacaaaaggcaatttattaaggaaatttgtaccatttcagtaaacctgtctgaaccggagagaccgagagagggtctcagttttataaagagtttgccttataaatttacataaaaatgtccgtttgtgtcttttgttg

SEQ ID NO: 43 - DNA, 2263 bp, synthetic construct
  source 1..2263: mol_type = other DNA
ataggcgccaagagcctagacttccttaagcgccagagtccacaagggcccagttaatcctcaacattcaaatgctgcccacaaaaccagcccctctgtgccctagccgcctcttttttccaagtgacagtagaactccaccaatccgcagctgaatggggtccgcctcttttccctgcctaaacagacaggaactcctgccaattgagggcgtcaccgctaaggctccgccccagcctgggctccacaaccaatgaagggtaatctcgacaaagagcaaggggtggggcgcgggcgcgcaggtgcagcagcacacaggctggtcgggagggcggggcgcgacgtctgccgtgcggggtcccggcatcggttgcgcgcgcgctccctcctctcggagagagggctgtggtaaaacccgtccggaaaccatggccgccgccgccgccgccgcgccgagcggaggaggaggaggaggcgaggaggagagactggaagaaaagtcagaagaccaggacctccagggcctcaaggacaaacccctcaagtttaaaaaggtgaagaaagataagaaagaagagaaagagggcaagcatgagcccgtgcagccatcagcccaccactctgctgagcccgcagaggcaggcaaagcagagacatcagaagggtcaggctccgccccggctgtgccggaagcttctgcctcccccaaacagcggcgctccatcatccgtgaccggggacccatgtatgatgaccccaccctgcctgaaggctggacacggaagcttaagcaaaggaaatctggccgctctgctgggaagtatgatgtgtatttgatcaatccccagggaaaagcctttcgctctaaagtggagttgattgcgtacttcgaaaaggtaggcgacacatccctggaccctaatgattttgacttcacggtaactgggagagggagcccctcccggcgagagcagaaaccacctaagaagcccaaatctcccaaagctccaggaactggcagaggccggggacgccccaaagggagcggcaccacgagacccaaggcggccacgtcagagggtgtgcaggtgaaaagggtcctggagaaaagtcctgggaagctccttgtcaagatgccttttcaaacttcgccagggggcaaggctgaggggggtggggccaccacatccacccaggtcatggtgatcaaacgccccggcaggaagcgaaaagctgaggccgaccctcaggccattcccaagaaacggggccgaaagccggggagtgtggtggcagccgctgccgccgaggccaaaaagaaagccgtgaaggagtcttctatccgatctgtgcaggagaccgtactccccatcaagaagcgcaagacccgggagacggtcagcatcgaggtcaaggaagtggtgaagcccctgctggtgtccaccctcggtgagaagagcgggaaaggactgaagacctgtaagagccctgggcggaaaagcaaggagagcagccccaaggggcgcagcagcagcgcctcctcaccccccaagaaggagcaccaccaccatcaccaccactcagagtccccaaaggcccccgtgccactgctcccacccctgcccccacctccacctgagcccgagagctccgaggaccccaccagcccccctgagccccaggacttgagcagcagcgtctgcaaagaggagaagatgcccagaggaggctcactggagagcgacggctgccccaaggagccagctaagactcagcccgcggttgccaccgccgccacggccgcagaaaagtacaaacaccgaggggagggagagcgcaaagacattgtttcatcctccatgccaaggccaaacagagaggagcctgtggacagccggacgcccgtgaccgagagagttagcgggagctccggcagttctggagaacaaaaactcatctcagaagaggatctgtgaacaagaataaaggcagctgttgtctcttctccttatgggtagggctctgacaaagcttcccatatcaccaggactgttaatatatttaaaaacaaaaggcaatttattaaggaaatttgtaccagtgaattctaccagtgccatagtacctgtatacgtttcaaaaactcccttctttcctcccgtctacaccccccccccactgaatccaaacaccattgtcacactccatataaagagtttgccttataaatttacataaaaatgtccgtttgtgtcttttgttg

SEQ ID NO: 44 - DNA, 2303 bp, synthetic construct
  source 1..2303: mol_type = other DNA
ataggcgccaagagcctagacttccttaagcgccagagtccacaagggcccagttaatcctcaacattcaaatgctgcccacaaaaccagcccctctgtgccctagccgcctcttttttccaagtgacagtagaactccaccaatccgcagctgaatggggtccgcctcttttccctgcctaaacagacaggaactcctgccaattgagggcgtcaccgctaaggctccgccccagcctgggctccacaaccaatgaagggtaatctcgacaaagagcaaggggtggggcgcgggcgcgcaggtgcagcagcacacaggctggtcgggagggcggggcgcgacgtctgccgtgcggggtcccggcatcggttgcgcgcgcgctccctcctctcggagagagggctgtggtaaaacccgtccggaaaccatggccgccgccgccgccgccgcgccgagcggaggaggaggaggaggcgaggaggagagactggaagaaaagtcagaagaccaggacctccagggcctcaaggacaaacccctcaagtttaaaaaggtgaagaaagataagaaagaagagaaagagggcaagcatgagcccgtgcagccatcagcccaccactctgctgagcccgcagaggcaggcaaagcagagacatcagaagggtcaggctccgccccggctgtgccggaagcttctgcctcccccaaacagcggcgctccatcatccgtgaccggggacccatgtatgatgaccccaccctgcctgaaggctggacacggaagcttaagcaaaggaaatctggccgctctgctgggaagtatgatgtgtatttgatcaatccccagggaaaagcctttcgctctaaagtggagttgattgcgtacttcgaaaaggtaggcgacacatccctggaccctaatgattttgacttcacggtaactgggagagggagcccctcccggcgagagcagaaaccacctaagaagcccaaatctcccaaagctccaggaactggcagaggccggggacgccccaaagggagcggcaccacgagacccaaggcggccacgtcagagggtgtgcaggtgaaaagggtcctggagaaaagtcctgggaagctccttgtcaagatgccttttcaaacttcgccagggggcaaggctgaggggggtggggccaccacatccacccaggtcatggtgatcaaacgccccggcaggaagcgaaaagctgaggccgaccctcaggccattcccaagaaacggggccgaaagccggggagtgtggtggcagccgctgccgccgaggccaaaaagaaagccgtgaaggagtcttctatccgatctgtgcaggagaccgtactccccatcaagaagcgcaagacccgggagacggtcagcatcgaggtcaaggaagtggtgaagcccctgctggtgtccaccctcggtgagaagagcgggaaaggactgaagacctgtaagagccctgggcggaaaagcaaggagagcagccccaaggggcgcagcagcagcgcctcctcaccccccaagaaggagcaccaccaccatcaccaccactcagagtccccaaaggcccccgtgccactgctcccacccctgcccccacctccacctgagcccgagagctccgaggaccccaccagcccccctgagccccaggacttgagcagcagcgtctgcaaagaggagaagatgcccagaggaggctcactggagagcgacggctgccccaaggagccagctaagactcagcccgcggttgccaccgccgccacggccgcagaaaagtacaaacaccgaggggagggagagcgcaaagacattgtttcatcctccatgccaaggccaaacagagaggagcctgtggacagccggacgcccgtgaccgagagagttagcgggagctccggcagttctggagaacaaaaactcatctcagaagaggatctgtgaacaagaataaaggcagctgttgtctcttctccttatgggtagggctctgacaaagcttcccatatcaccaggactgttaatatatttaaaaacaaaaggcaatttattaaggaaatttgtaccagtgaattctaccagtgccatagtacctgtatacgtttcaaaaactcccttctttcctcccgtctacaccccccccccactgaatccaaacaccattgtcacactccacctgtaacctatttattattggcattcaccgcgtgccttatataaagagtttgccttataaatttacataaaaatgtccgtttgtgtcttttgttg

SEQ ID NO: 45 - DNA, 2303 bp, synthetic construct
  source 1..2303: mol_type = other DNA
ataggcgccaagagcctagacttccttaagcgccagagtccacaagggcccagttaatcctcaacattcaaatgctgcccacaaaaccagcccctctgtgccctagccgcctcttttttccaagtgacagtagaactccaccaatccgcagctgaatggggtccgcctcttttccctgcctaaacagacaggaactcctgccaattgagggcgtcaccgctaaggctccgccccagcctgggctccacaaccaatgaagggtaatctcgacaaagagcaaggggtggggcgcgggcgcgcaggtgcagcagcacacaggctggtcgggagggcggggcgcgacgtctgccgtgcggggtcccggcatcggttgcgcgcgcgctccctcctctcggagagagggctgtggtaaaacccgtccggaaaccatggccgccgccgccgccgccgcgccgagcggaggaggaggaggaggcgaggaggagagactggaagaaaagtcagaagaccaggacctccagggcctcaaggacaaacccctcaagtttaaaaaggtgaagaaagataagaaagaagagaaagagggcaagcatgagcccgtgcagccatcagcccaccactctgctgagcccgcagaggcaggcaaagcagagacatcagaagggtcaggctccgccccggctgtgccggaagcttctgcctcccccaaacagcggcgctccatcatccgtgaccggggacccatgtatgatgaccccaccctgcctgaaggctggacacggaagcttaagcaaaggaaatctggccgctctgctgggaagtatgatgtgtatttgatcaatccccagggaaaagcctttcgctctaaagtggagttgattgcgtacttcgaaaaggtaggcgacacatccctggaccctaatgattttgacttcacggtaactgggagagggagcccctcccggcgagagcagaaaccacctaagaagcccaaatctcccaaagctccaggaactggcagaggccggggacgccccaaagggagcggcaccacgagacccaaggcggccacgtcagagggtgtgcaggtgaaaagggtcctggagaaaagtcctgggaagctccttgtcaagatgccttttcaaacttcgccagggggcaaggctgaggggggtggggccaccacatccacccaggtcatggtgatcaaacgccccggcaggaagcgaaaagctgaggccgaccctcaggccattcccaagaaacggggccgaaagccggggagtgtggtggcagccgctgccgccgaggccaaaaagaaagccgtgaaggagtcttctatccgatctgtgcaggagaccgtactccccatcaagaagcgcaagacccgggagacggtcagcatcgaggtcaaggaagtggtgaagcccctgctggtgtccaccctcggtgagaagagcgggaaaggactgaagacctgtaagagccctgggcggaaaagcaaggagagcagccccaaggggcgcagcagcagcgcctcctcaccccccaagaaggagcaccaccaccatcaccaccactcagagtccccaaaggcccccgtgccactgctcccacccctgcccccacctccacctgagcccgagagctccgaggaccccaccagcccccctgagccccaggacttgagcagcagcgtctgcaaagaggagaagatgcccagaggaggctcactggagagcgacggctgccccaaggagccagctaagactcagcccgcggttgccaccgccgccacggccgcagaaaagtacaaacaccgaggggagggagagcgcaaagacattgtttcatcctccatgccaaggccaaacagagaggagcctgtggacagccggacgcccgtgaccgagagagttagcgggagctccggcagttctggagaacaaaaactcatctcagaagaggatctgtgaacaagaataaaggcagctgttgtctcttctccttatgggtagggctctgacaaagcttcccatatcaccaggactgttaatatatttaaaaacaaaaggcaatttattaaggaaatttgtaccagtgaattctaccagtgccatagtacctgtatacgtttcaaaaactcccttctttcctcccgtctacaccccccccccactgaatccaaacaccattgtcacactccacctgtaacctatttattaatgcccttttaacattgcactatataaagagtttgccttataaatttacataaaaatgtccgtttgtgtcttttgttg

SEQ ID NO: 46 - DNA, 2303 bp, synthetic construct
  source 1..2303: mol_type = other DNA
ataggcgccaagagcctagacttccttaagcgccagagtccacaagggcccagttaatcctcaacattcaaatgctgcccacaaaaccagcccctctgtgccctagccgcctcttttttccaagtgacagtagaactccaccaatccgcagctgaatggggtccgcctcttttccctgcctaaacagacaggaactcctgccaattgagggcgtcaccgctaaggctccgccccagcctgggctccacaaccaatgaagggtaatctcgacaaagagcaaggggtggggcgcgggcgcgcaggtgcagcagcacacaggctggtcgggagggcggggcgcgacgtctgccgtgcggggtcccggcatcggttgcgcgcgcgctccctcctctcggagagagggctgtggtaaaacccgtccggaaaccatggccgccgccgccgccgccgcgccgagcggaggaggaggaggaggcgaggaggagagactggaagaaaagtcagaagaccaggacctccagggcctcaaggacaaacccctcaagtttaaaaaggtgaagaaagataagaaagaagagaaagagggcaagcatgagcccgtgcagccatcagcccaccactctgctgagcccgcagaggcaggcaaagcagagacatcagaagggtcaggctccgccccggctgtgccggaagcttctgcctcccccaaacagcggcgctccatcatccgtgaccggggacccatgtatgatgaccccaccctgcctgaaggctggacacggaagcttaagcaaaggaaatctggccgctctgctgggaagtatgatgtgtatttgatcaatccccagggaaaagcctttcgctctaaagtggagttgattgcgtacttcgaaaaggtaggcgacacatccctggaccctaatgattttgacttcacggtaactgggagagggagcccctcccggcgagagcagaaaccacctaagaagcccaaatctcccaaagctccaggaactggcagaggccggggacgccccaaagggagcggcaccacgagacccaaggcggccacgtcagagggtgtgcaggtgaaaagggtcctggagaaaagtcctgggaagctccttgtcaagatgccttttcaaacttcgccagggggcaaggctgaggggggtggggccaccacatccacccaggtcatggtgatcaaacgccccggcaggaagcgaaaagctgaggccgaccctcaggccattcccaagaaacggggccgaaagccggggagtgtggtggcagccgctgccgccgaggccaaaaagaaagccgtgaaggagtcttctatccgatctgtgcaggagaccgtactccccatcaagaagcgcaagacccgggagacggtcagcatcgaggtcaaggaagtggtgaagcccctgctggtgtccaccctcggtgagaagagcgggaaaggactgaagacctgtaagagccctgggcggaaaagcaaggagagcagccccaaggggcgcagcagcagcgcctcctcaccccccaagaaggagcaccaccaccatcaccaccactcagagtccccaaaggcccccgtgccactgctcccacccctgcccccacctccacctgagcccgagagctccgaggaccccaccagcccccctgagccccaggacttgagcagcagcgtctgcaaagaggagaagatgcccagaggaggctcactggagagcgacggctgccccaaggagccagctaagactcagcccgcggttgccaccgccgccacggccgcagaaaagtacaaacaccgaggggagggagagcgcaaagacattgtttcatcctccatgccaaggccaaacagagaggagcctgtggacagccggacgcccgtgaccgagagagttagcgggagctccggcagttctggagaacaaaaactcatctcagaagaggatctgtgaacaagaataaaggcagctgttgtctcttctccttatgggtagggctctgacaaagcttcccatatcaccaggactgttaatatatttaaaaacaaaaggcaatttattaaggaaatttgtaccagtgaattctaccagtgccatagtacctgtatacgtttcaaaaactcccttctttcctcccgtctacaccccccccccactgaatccaaacaccattgtcacactccacctgtaacctatttattacgaccatggctgtagactgttatataaagagtttgccttataaatttacataaaaatgtccgtttgtgtcttttgttg

SEQ ID NO: 47 - DNA, 2101 bp, synthetic construct
  source 1..2101: mol_type = other DNA
agccgcctcttttttccaagtgacagtagaactccaccaatccgcagctgaatggggtccgcctcttttccctgcctaaacagacaggaactcctgccaattgagggcgtcaccgctaaggctccgccccagcctgggctccacaaccaatgaagggtaatctcgacaaagagcaaggggtggggcgcgggcgcgcaggtgcagcagcacacaggctggtcgggagggcggggcgcgacgtctgccgtgcggggtcccggcatcggttgcgcgcgcgctccctcctctcggagagagggctgtggtaaaacccgtccggaaaccatggccgccgccgccgccgccgcgccgagcggaggaggaggaggaggcgaggaggagagactggaagaaaagtcagaagaccaggacctccagggcctcaaggacaaacccctcaagtttaaaaaggtgaagaaagataagaaagaagagaaagagggcaagcatgagcccgtgcagccatcagcccaccactctgctgagcccgcagaggcaggcaaagcagagacatcagaagggtcaggctccgccccggctgtgccggaagcttctgcctcccccaaacagcggcgctccatcatccgtgaccggggacccatgtatgatgaccccaccctgcctgaaggctggacacggaagcttaagcaaaggaaatctggccgctctgctgggaagtatgatgtgtatttgatcaatccccagggaaaagcctttcgctctaaagtggagttgattgcgtacttcgaaaaggtaggcgacacatccctggaccctaatgattttgacttcacggtaactgggagagggagcccctcccggcgagagcagaaaccacctaagaagcccaaatctcccaaagctccaggaactggcagaggccggggacgccccaaagggagcggcaccacgagacccaaggcggccacgtcagagggtgtgcaggtgaaaagggtcctggagaaaagtcctgggaagctccttgtcaagatgccttttcaaacttcgccagggggcaaggctgaggggggtggggccaccacatccacccaggtcatggtgatcaaacgccccggcaggaagcgaaaagctgaggccgaccctcaggccattcccaagaaacggggccgaaagccggggagtgtggtggcagccgctgccgccgaggccaaaaagaaagccgtgaaggagtcttctatccgatctgtgcaggagaccgtactccccatcaagaagcgcaagacccgggagacggtcagcatcgaggtcaaggaagtggtgaagcccctgctggtgtccaccctcggtgagaagagcgggaaaggactgaagacctgtaagagccctgggcggaaaagcaaggagagcagccccaaggggcgcagcagcagcgcctcctcaccccccaagaaggagcaccaccaccatcaccaccactcagagtccccaaaggcccccgtgccactgctcccacccctgcccccacctccacctgagcccgagagctccgaggaccccaccagcccccctgagccccaggacttgagcagcagcgtctgcaaagaggagaagatgcccagaggaggctcactggagagcgacggctgccccaaggagccagctaagactcagcccgcggttgccaccgccgccacggccgcagaaaagtacaaacaccgaggggagggagagcgcaaagacattgtttcatcctccatgccaaggccaaacagagaggagcctgtggacagccggacgcccgtgaccgagagagttagcgggagctccggcagttctggagaacaaaaactcatctcagaagaggatctgtgaacaagaataaaggcagctgttgtctcttctccttatgggtagggctctgacaaagcttcccatatcaccaggactgttaatatatttaaaaacaaaaggcaatttattaaggaaatttgtaccatttcagtaaacctgtctgaaccggagagaccgagagagggtctcagttttataaagagtttgccttataaatttacataaaaatgtccgtttgtgtcttttgttg

SEQ ID NO: 48 - DNA, 2159 bp, synthetic construct
  source 1..2159: mol_type = other DNA
agccgcctcttttttccaagtgacagtagaactccaccaatccgcagctgaatggggtccgcctcttttccctgcctaaacagacaggaactcctgccaattgagggcgtcaccgctaaggctccgccccagcctgggctccacaaccaatgaagggtaatctcgacaaagagcaaggggtggggcgcgggcgcgcaggtgcagcagcacacaggctggtcgggagggcggggcgcgacgtctgccgtgcggggtcccggcatcggttgcgcgcgcgctccctcctctcggagagagggctgtggtaaaacccgtccggaaaccatggccgccgccgccgccgccgcgccgagcggaggaggaggaggaggcgaggaggagagactggaagaaaagtcagaagaccaggacctccagggcctcaaggacaaacccctcaagtttaaaaaggtgaagaaagataagaaagaagagaaagagggcaagcatgagcccgtgcagccatcagcccaccactctgctgagcccgcagaggcaggcaaagcagagacatcagaagggtcaggctccgccccggctgtgccggaagcttctgcctcccccaaacagcggcgctccatcatccgtgaccggggacccatgtatgatgaccccaccctgcctgaaggctggacacggaagcttaagcaaaggaaatctggccgctctgctgggaagtatgatgtgtatttgatcaatccccagggaaaagcctttcgctctaaagtggagttgattgcgtacttcgaaaaggtaggcgacacatccctggaccctaatgattttgacttcacggtaactgggagagggagcccctcccggcgagagcagaaaccacctaagaagcccaaatctcccaaagctccaggaactggcagaggccggggacgccccaaagggagcggcaccacgagacccaaggcggccacgtcagagggtgtgcaggtgaaaagggtcctggagaaaagtcctgggaagctccttgtcaagatgccttttcaaacttcgccagggggcaaggctgaggggggtggggccaccacatccacccaggtcatggtgatcaaacgccccggcaggaagcgaaaagctgaggccgaccctcaggccattcccaagaaacggggccgaaagccggggagtgtggtggcagccgctgccgccgaggccaaaaagaaagccgtgaaggagtcttctatccgatctgtgcaggagaccgtactccccatcaagaagcgcaagacccgggagacggtcagcatcgaggtcaaggaagtggtgaagcccctgctggtgtccaccctcggtgagaagagcgggaaaggactgaagacctgtaagagccctgggcggaaaagcaaggagagcagccccaaggggcgcagcagcagcgcctcctcaccccccaagaaggagcaccaccaccatcaccaccactcagagtccccaaaggcccccgtgccactgctcccacccctgcccccacctccacctgagcccgagagctccgaggaccccaccagcccccctgagccccaggacttgagcagcagcgtctgcaaagaggagaagatgcccagaggaggctcactggagagcgacggctgccccaaggagccagctaagactcagcccgcggttgccaccgccgccacggccgcagaaaagtacaaacaccgaggggagggagagcgcaaagacattgtttcatcctccatgccaaggccaaacagagaggagcctgtggacagccggacgcccgtgaccgagagagttagcgggagctccggcagttctggagaacaaaaactcatctcagaagaggatctgtgaacaagaataaaggcagctgttgtctcttctccttatgggtagggctctgacaaagcttcccatatcaccaggactgttaatatatttaaaaacaaaaggcaatttattaaggaaatttgtaccagtgaattctaccagtgccatagtacctgtatacgtttcaaaaactcccttctttcctcccgtctacaccccccccccactgaatccaaacaccattgtcacactccatataaagagtttgccttataaatttacataaaaatgtccgtttgtgtcttttgttg

SEQ ID NO: 49 - DNA, 2199 bp, synthetic construct
  source 1..2199: mol_type = other DNA
agccgcctcttttttccaagtgacagtagaactccaccaatccgcagctgaatggggtccgcctcttttccctgcctaaacagacaggaactcctgccaattgagggcgtcaccgctaaggctccgccccagcctgggctccacaaccaatgaagggtaatctcgacaaagagcaaggggtggggcgcgggcgcgcaggtgcagcagcacacaggctggtcgggagggcggggcgcgacgtctgccgtgcggggtcccggcatcggttgcgcgcgcgctccctcctctcggagagagggctgtggtaaaacccgtccggaaaccatggccgccgccgccgccgccgcgccgagcggaggaggaggaggaggcgaggaggagagactggaagaaaagtcagaagaccaggacctccagggcctcaaggacaaacccctcaagtttaaaaaggtgaagaaagataagaaagaagagaaagagggcaagcatgagcccgtgcagccatcagcccaccactctgctgagcccgcagaggcaggcaaagcagagacatcagaagggtcaggctccgccccggctgtgccggaagcttctgcctcccccaaacagcggcgctccatcatccgtgaccggggacccatgtatgatgaccccaccctgcctgaaggctggacacggaagcttaagcaaaggaaatctggccgctctgctgggaagtatgatgtgtatttgatcaatccccagggaaaagcctttcgctctaaagtggagttgattgcgtacttcgaaaaggtaggcgacacatccctggaccctaatgattttgacttcacggtaactgggagagggagcccctcccggcgagagcagaaaccacctaagaagcccaaatctcccaaagctccaggaactggcagaggccggggacgccccaaagggagcggcaccacgagacccaaggcggccacgtcagagggtgtgcaggtgaaaagggtcctggagaaaagtcctgggaagctccttgtcaagatgccttttcaaacttcgccagggggcaaggctgaggggggtggggccaccacatccacccaggtcatggtgatcaaacgccccggcaggaagcgaaaagctgaggccgaccctcaggccattcccaagaaacggggccgaaagccggggagtgtggtggcagccgctgccgccgaggccaaaaagaaagccgtgaaggagtcttctatccgatctgtgcaggagaccgtactccccatcaagaagcgcaagacccgggagacggtcagcatcgaggtcaaggaagtggtgaagcccctgctggtgtccaccctcggtgagaagagcgggaaaggactgaagacctgtaagagccctgggcggaaaagcaaggagagcagccccaaggggcgcagcagcagcgcctcctcaccccccaagaaggagcaccaccaccatcaccaccactcagagtccccaaaggcccccgtgccactgctcccacccctgcccccacctccacctgagcccgagagctccgaggaccccaccagcccccctgagccccaggacttgagcagcagcgtctgcaaagaggagaagatgcccagaggaggctcactggagagcgacggctgccccaaggagccagctaagactcagcccgcggttgccaccgccgccacggccgcagaaaagtacaaacaccgaggggagggagagcgcaaagacattgtttcatcctccatgccaaggccaaacagagaggagcctgtggacagccggacgcccgtgaccgagagagttagcgggagctccggcagttctggagaacaaaaactcatctcagaagaggatctgtgaacaagaataaaggcagctgttgtctcttctccttatgggtagggctctgacaaagcttcccatatcaccaggactgttaatatatttaaaaacaaaaggcaatttattaaggaaatttgtaccagtgaattctaccagtgccatagtacctgtatacgtttcaaaaactcccttctttcctcccgtctacaccccccccccactgaatccaaacaccattgtcacactccacctgtaacctatttattattggcattcaccgcgtgccttatataaagagtttgccttataaatttacataaaaatgtccgtttgtgtcttttgttg

SEQ ID NO: 50 - DNA, 2154 bp, synthetic construct
  source 1..2154: mol_type = other DNA
agctgaatggggtccgcctcttttccctgcctaaacagacaggaactcctgccaattgagggcgtcaccgctaaggctccgccccagcctgggctccacaaccaatgaagggtaatctcgacaaagagcaaggggtggggcgcgggcgcgcaggtgcagcagcacacaggctggtcgggagggcggggcgcgacgtctgccgtgcggggtcccggcatcggttgcgcgcgcgctccctcctctcggagagagggctgtggtaaaacccgtccggaaaccatggccgccgccgccgccgccgcgccgagcggaggaggaggaggaggcgaggaggagagactggaagaaaagtcagaagaccaggacctccagggcctcaaggacaaacccctcaagtttaaaaaggtgaagaaagataagaaagaagagaaagagggcaagcatgagcccgtgcagccatcagcccaccactctgctgagcccgcagaggcaggcaaagcagagacatcagaagggtcaggctccgccccggctgtgccggaagcttctgcctcccccaaacagcggcgctccatcatccgtgaccggggacccatgtatgatgaccccaccctgcctgaaggctggacacggaagcttaagcaaaggaaatctggccgctctgctgggaagtatgatgtgtatttgatcaatccccagggaaaagcctttcgctctaaagtggagttgattgcgtacttcgaaaaggtaggcgacacatccctggaccctaatgattttgacttcacggtaactgggagagggagcccctcccggcgagagcagaaaccacctaagaagcccaaatctcccaaagctccaggaactggcagaggccggggacgccccaaagggagcggcaccacgagacccaaggcggccacgtcagagggtgtgcaggtgaaaagggtcctggagaaaagtcctgggaagctccttgtcaagatgccttttcaaacttcgccagggggcaaggctgaggggggtggggccaccacatccacccaggtcatggtgatcaaacgccccggcaggaagcgaaaagctgaggccgaccctcaggccattcccaagaaacggggccgaaagccggggagtgtggtggcagccgctgccgccgaggccaaaaagaaagccgtgaaggagtcttctatccgatctgtgcaggagaccgtactccccatcaagaagcgcaagacccgggagacggtcagcatcgaggtcaaggaagtggtgaagcccctgctggtgtccaccctcggtgagaagagcgggaaaggactgaagacctgtaagagccctgggcggaaaagcaaggagagcagccccaaggggcgcagcagcagcgcctcctcaccccccaagaaggagcaccaccaccatcaccaccactcagagtccccaaaggcccccgtgccactgctcccacccctgcccccacctccacctgagcccgagagctccgaggaccccaccagcccccctgagccccaggacttgagcagcagcgtctgcaaagaggagaagatgcccagaggaggctcactggagagcgacggctgccccaaggagccagctaagactcagcccgcggttgccaccgccgccacggccgcagaaaagtacaaacaccgaggggagggagagcgcaaagacattgtttcatcctccatgccaaggccaaacagagaggagcctgtggacagccggacgcccgtgaccgagagagttagcgggagctccggcagttctggagaacaaaaactcatctcagaagaggatctgtgaacaagaataaaggcagctgttgtctcttctccttatgggtagggctctgacaaagcttcccatatcaccaggactgttaatatatttaaaaacaaaaggcaatttattaaggaaatttgtaccagtgaattctaccagtgccatagtacctgtatacgtttcaaaaactcccttctttcctcccgtctacaccccccccccactgaatccaaacaccattgtcacactccacctgtaacctatttattaatgcccttttaacattgcactatataaagagtttgccttataaatttacataaaaatgtccgtttgtgtcttttgttg

SEQ ID NO: 51 - DNA, 2199 bp, synthetic construct
  source 1..2199: mol_type = other DNA
agccgcctcttttttccaagtgacagtagaactccaccaatccgcagctgaatggggtccgcctcttttccctgcctaaacagacaggaactcctgccaattgagggcgtcaccgctaaggctccgccccagcctgggctccacaaccaatgaagggtaatctcgacaaagagcaaggggtggggcgcgggcgcgcaggtgcagcagcacacaggctggtcgggagggcggggcgcgacgtctgccgtgcggggtcccggcatcggttgcgcgcgcgctccctcctctcggagagagggctgtggtaaaacccgtccggaaaccatggccgccgccgccgccgccgcgccgagcggaggaggaggaggaggcgaggaggagagactggaagaaaagtcagaagaccaggacctccagggcctcaaggacaaacccctcaagtttaaaaaggtgaagaaagataagaaagaagagaaagagggcaagcatgagcccgtgcagccatcagcccaccactctgctgagcccgcagaggcaggcaaagcagagacatcagaagggtcaggctccgccccggctgtgccggaagcttctgcctcccccaaacagcggcgctccatcatccgtgaccggggacccatgtatgatgaccccaccctgcctgaaggctggacacggaagcttaagcaaaggaaatctggccgctctgctgggaagtatgatgtgtatttgatcaatccccagggaaaagcctttcgctctaaagtggagttgattgcgtacttcgaaaaggtaggcgacacatccctggaccctaatgattttgacttcacggtaactgggagagggagcccctcccggcgagagcagaaaccacctaagaagcccaaatctcccaaagctccaggaactggcagaggccggggacgccccaaagggagcggcaccacgagacccaaggcggccacgtcagagggtgtgcaggtgaaaagggtcctggagaaaagtcctgggaagctccttgtcaagatgccttttcaaacttcgccagggggcaaggctgaggggggtggggccaccacatccacccaggtcatggtgatcaaacgccccggcaggaagcgaaaagctgaggccgaccctcaggccattcccaagaaacggggccgaaagccggggagtgtggtggcagccgctgccgccgaggccaaaaagaaagccgtgaaggagtcttctatccgatctgtgcaggagaccgtactccccatcaagaagcgcaagacccgggagacggtcagcatcgaggtcaaggaagtggtgaagcccctgctggtgtccaccctcggtgagaagagcgggaaaggactgaagacctgtaagagccctgggcggaaaagcaaggagagcagccccaaggggcgcagcagcagcgcctcctcaccccccaagaaggagcaccaccaccatcaccaccactcagagtccccaaaggcccccgtgccactgctcccacccctgcccccacctccacctgagcccgagagctccgaggaccccaccagcccccctgagccccaggacttgagcagcagcgtctgcaaagaggagaagatgcccagaggaggctcactggagagcgacggctgccccaaggagccagctaagactcagcccgcggttgccaccgccgccacggccgcagaaaagtacaaacaccgaggggagggagagcgcaaagacattgtttcatcctccatgccaaggccaaacagagaggagcctgtggacagccggacgcccgtgaccgagagagttagcgggagctccggcagttctggagaacaaaaactcatctcagaagaggatctgtgaacaagaataaaggcagctgttgtctcttctccttatgggtagggctctgacaaagcttcccatatcaccaggactgttaatatatttaaaaacaaaaggcaatttattaaggaaatttgtaccagtgaattctaccagtgccatagtacctgtatacgtttcaaaaactcccttctttcctcccgtctacaccccccccccactgaatccaaacaccattgtcacactccacctgtaacctatttattacgaccatggctgtagactgttatataaagagtttgccttataaatttacataaaaatgtccgtttgtgtcttttgttg

SEQ ID NO: 52 - DNA, 2002 bp, synthetic construct
  source 1..2002: mol_type = other DNA
attgagggcgtcaccgctaaggctccgccccagcctgggctccacaaccaatgaagggtaatctcgacaaagagcaaggggtggggcgcgggcgcgcaggtgcagcagcacacaggctggtcgggagggcggggcgcgacgtctgccgtgcggggtcccggcatcggttgcgcgcgcgctccctcctctcggagagagggctgtggtaaaacccgtccggaaaccatggccgccgccgccgccgccgcgccgagcggaggaggaggaggaggcgaggaggagagactggaagaaaagtcagaagaccaggacctccagggcctcaaggacaaacccctcaagtttaaaaaggtgaagaaagataagaaagaagagaaagagggcaagcatgagcccgtgcagccatcagcccaccactctgctgagcccgcagaggcaggcaaagcagagacatcagaagggtcaggctccgccccggctgtgccggaagcttctgcctcccccaaacagcggcgctccatcatccgtgaccggggacccatgtatgatgaccccaccctgcctgaaggctggacacggaagcttaagcaaaggaaatctggccgctctgctgggaagtatgatgtgtatttgatcaatccccagggaaaagcctttcgctctaaagtggagttgattgcgtacttcgaaaaggtaggcgacacatccctggaccctaatgattttgacttcacggtaactgggagagggagcccctcccggcgagagcagaaaccacctaagaagcccaaatctcccaaagctccaggaactggcagaggccggggacgccccaaagggagcggcaccacgagacccaaggcggccacgtcagagggtgtgcaggtgaaaagggtcctggagaaaagtcctgggaagctccttgtcaagatgccttttcaaacttcgccagggggcaaggctgaggggggtggggccaccacatccacccaggtcatggtgatcaaacgccccggcaggaagcgaaaagctgaggccgaccctcaggccattcccaagaaacggggccgaaagccggggagtgtggtggcagccgctgccgccgaggccaaaaagaaagccgtgaaggagtcttctatccgatctgtgcaggagaccgtactccccatcaagaagcgcaagacccgggagacggtcagcatcgaggtcaaggaagtggtgaagcccctgctggtgtccaccctcggtgagaagagcgggaaaggactgaagacctgtaagagccctgggcggaaaagcaaggagagcagccccaaggggcgcagcagcagcgcctcctcaccccccaagaaggagcaccaccaccatcaccaccactcagagtccccaaaggcccccgtgccactgctcccacccctgcccccacctccacctgagcccgagagctccgaggaccccaccagcccccctgagccccaggacttgagcagcagcgtctgcaaagaggagaagatgcccagaggaggctcactggagagcgacggctgccccaaggagccagctaagactcagcccgcggttgccaccgccgccacggccgcagaaaagtacaaacaccgaggggagggagagcgcaaagacattgtttcatcctccatgccaaggccaaacagagaggagcctgtggacagccggacgcccgtgaccgagagagttagcgggagctccggcagttctggagaacaaaaactcatctcagaagaggatctgtgaacaagaataaaggcagctgttgtctcttctccttatgggtagggctctgacaaagcttcccatatcaccaggactgttaatatatttaaaaacaaaaggcaatttattaaggaaatttgtaccatttcagtaaacctgtctgaaccggagagaccgagagagggtctcagttttataaagagtttgccttataaatttacataaaaatgtccgtttgtgtcttttgttg

SEQ ID NO: 53 - DNA, 2060 bp, synthetic construct
  source 1..2060: mol_type = other DNA
attgagggcgtcaccgctaaggctccgccccagcctgggctccacaaccaatgaagggtaatctcgacaaagagcaaggggtggggcgcgggcgcgcaggtgcagcagcacacaggctggtcgggagggcggggcgcgacgtctgccgtgcggggtcccggcatcggttgcgcgcgcgctccctcctctcggagagagggctgtggtaaaacccgtccggaaaccatggccgccgccgccgccgccgcgccgagcggaggaggaggaggaggcgaggaggagagactggaagaaaagtcagaagaccaggacctccagggcctcaaggacaaacccctcaagtttaaaaaggtgaagaaagataagaaagaagagaaagagggcaagcatgagcccgtgcagccatcagcccaccactctgctgagcccgcagaggcaggcaaagcagagacatcagaagggtcaggctccgccccggctgtgccggaagcttctgcctcccccaaacagcggcgctccatcatccgtgaccggggacccatgtatgatgaccccaccctgcctgaaggctggacacggaagcttaagcaaaggaaatctggccgctctgctgggaagtatgatgtgtatttgatcaatccccagggaaaagcctttcgctctaaagtggagttgattgcgtacttcgaaaaggtaggcgacacatccctggaccctaatgattttgacttcacggtaactgggagagggagcccctcccggcgagagcagaaaccacctaagaagcccaaatctcccaaagctccaggaactggcagaggccggggacgccccaaagggagcggcaccacgagacccaaggcggccacgtcagagggtgtgcaggtgaaaagggtcctggagaaaagtcctgggaagctccttgtcaagatgccttttcaaacttcgccagggggcaaggctgaggggggtggggccaccacatccacccaggtcatggtgatcaaacgccccggcaggaagcgaaaagctgaggccgaccctcaggccattcccaagaaacggggccgaaagccggggagtgtggtggcagccgctgccgccgaggccaaaaagaaagccgtgaaggagtcttctatccgatctgtgcaggagaccgtactccccatcaagaagcgcaagacccgggagacggtcagcatcgaggtcaaggaagtggtgaagcccctgctggtgtccaccctcggtgagaagagcgggaaaggactgaagacctgtaagagccctgggcggaaaagcaaggagagcagccccaaggggcgcagcagcagcgcctcctcaccccccaagaaggagcaccaccaccatcaccaccactcagagtccccaaaggcccccgtgccactgctcccacccctgcccccacctccacctgagcccgagagctccgaggaccccaccagcccccctgagccccaggacttgagcagcagcgtctgcaaagaggagaagatgcccagaggaggctcactggagagcgacggctgccccaaggagccagctaagactcagcccgcggttgccaccgccgccacggccgcagaaaagtacaaacaccgaggggagggagagcgcaaagacattgtttcatcctccatgccaaggccaaacagagaggagcctgtggacagccggacgcccgtgaccgagagagttagcgggagctccggcagttctggagaacaaaaactcatctcagaagaggatctgtgaacaagaataaaggcagctgttgtctcttctccttatgggtagggctctgacaaagcttcccatatcaccaggactgttaatatatttaaaaacaaaaggcaatttattaaggaaatttgtaccagtgaattctaccagtgccatagtacctgtatacgtttcaaaaactcccttctttcctcccgtctacaccccccccccactgaatccaaacaccattgtcacactccatataaagagtttgccttataaatttacataaaaatgtccgtttgtgtcttttgttg

SEQ ID NO: 54 - DNA, 2100 bp, synthetic construct
  source 1..2100: mol_type = other DNA
attgagggcgtcaccgctaaggctccgccccagcctgggctccacaaccaatgaagggtaatctcgacaaagagcaaggggtggggcgcgggcgcgcaggtgcagcagcacacaggctggtcgggagggcggggcgcgacgtctgccgtgcggggtcccggcatcggttgcgcgcgcgctccctcctctcggagagagggctgtggtaaaacccgtccggaaaccatggccgccgccgccgccgccgcgccgagcggaggaggaggaggaggcgaggaggagagactggaagaaaagtcagaagaccaggacctccagggcctcaaggacaaacccctcaagtttaaaaaggtgaagaaagataagaaagaagagaaagagggcaagcatgagcccgtgcagccatcagcccaccactctgctgagcccgcagaggcaggcaaagcagagacatcagaagggtcaggctccgccccggctgtgccggaagcttctgcctcccccaaacagcggcgctccatcatccgtgaccggggacccatgtatgatgaccccaccctgcctgaaggctggacacggaagcttaagcaaaggaaatctggccgctctgctgggaagtatgatgtgtatttgatcaatccccagggaaaagcctttcgctctaaagtggagttgattgcgtacttcgaaaaggtaggcgacacatccctggaccctaatgattttgacttcacggtaactgggagagggagcccctcccggcgagagcagaaaccacctaagaagcccaaatctcccaaagctccaggaactggcagaggccggggacgccccaaagggagcggcaccacgagacccaaggcggccacgtcagagggtgtgcaggtgaaaagggtcctggagaaaagtcctgggaagctccttgtcaagatgccttttcaaacttcgccagggggcaaggctgaggggggtggggccaccacatccacccaggtcatggtgatcaaacgccccggcaggaagcgaaaagctgaggccgaccctcaggccattcccaagaaacggggccgaaagccggggagtgtggtggcagccgctgccgccgaggccaaaaagaaagccgtgaaggagtcttctatccgatctgtgcaggagaccgtactccccatcaagaagcgcaagacccgggagacggtcagcatcgaggtcaaggaagtggtgaagcccctgctggtgtccaccctcggtgagaagagcgggaaaggactgaagacctgtaagagccctgggcggaaaagcaaggagagcagccccaaggggcgcagcagcagcgcctcctcaccccccaagaaggagcaccaccaccatcaccaccactcagagtccccaaaggcccccgtgccactgctcccacccctgcccccacctccacctgagcccgagagctccgaggaccccaccagcccccctgagccccaggacttgagcagcagcgtctgcaaagaggagaagatgcccagaggaggctcactggagagcgacggctgccccaaggagccagctaagactcagcccgcggttgccaccgccgccacggccgcagaaaagtacaaacaccgaggggagggagagcgcaaagacattgtttcatcctccatgccaaggccaaacagagaggagcctgtggacagccggacgcccgtgaccgagagagttagcgggagctccggcagttctggagaacaaaaactcatctcagaagaggatctgtgaacaagaataaaggcagctgttgtctcttctccttatgggtagggctctgacaaagcttcccatatcaccaggactgttaatatatttaaaaacaaaaggcaatttattaaggaaatttgtaccagtgaattctaccagtgccatagtacctgtatacgtttcaaaaactcccttctttcctcccgtctacaccccccccccactgaatccaaacaccattgtcacactccacctgtaacctatttattattggcattcaccgcgtgccttatataaagagtttgccttataaatttacataaaaatgtccgtttgtgtcttttgttg

SEQ ID NO: 55 - DNA, 2100 bp, synthetic construct
  source 1..2100: mol_type = other DNA
attgagggcgtcaccgctaaggctccgccccagcctgggctccacaaccaatgaagggtaatctcgacaaagagcaaggggtggggcgcgggcgcgcaggtgcagcagcacacaggctggtcgggagggcggggcgcgacgtctgccgtgcggggtcccggcatcggttgcgcgcgcgctccctcctctcggagagagggctgtggtaaaacccgtccggaaaccatggccgccgccgccgccgccgcgccgagcggaggaggaggaggaggcgaggaggagagactggaagaaaagtcagaagaccaggacctccagggcctcaaggacaaacccctcaagtttaaaaaggtgaagaaagataagaaagaagagaaagagggcaagcatgagcccgtgcagccatcagcccaccactctgctgagcccgcagaggcaggcaaagcagagacatcagaagggtcaggctccgccccggctgtgccggaagcttctgcctcccccaaacagcggcgctccatcatccgtgaccggggacccatgtatgatgaccccaccctgcctgaaggctggacacggaagcttaagcaaaggaaatctggccgctctgctgggaagtatgatgtgtatttgatcaatccccagggaaaagcctttcgctctaaagtggagttgattgcgtacttcgaaaaggtaggcgacacatccctggaccctaatgattttgacttcacggtaactgggagagggagcccctcccggcgagagcagaaaccacctaagaagcccaaatctcccaaagctccaggaactggcagaggccggggacgccccaaagggagcggcaccacgagacccaaggcggccacgtcagagggtgtgcaggtgaaaagggtcctggagaaaagtcctgggaagctccttgtcaagatgccttttcaaacttcgccagggggcaaggctgaggggggtggggccaccacatccacccaggtcatggtgatcaaacgccccggcaggaagcgaaaagctgaggccgaccctcaggccattcccaagaaacggggccgaaagccggggagtgtggtggcagccgctgccgccgaggccaaaaagaaagccgtgaaggagtcttctatccgatctgtgcaggagaccgtactccccatcaagaagcgcaagacccgggagacggtcagcatcgaggtcaaggaagtggtgaagcccctgctggtgtccaccctcggtgagaagagcgggaaaggactgaagacctgtaagagccctgggcggaaaagcaaggagagcagccccaaggggcgcagcagcagcgcctcctcaccccccaagaaggagcaccaccaccatcaccaccactcagagtccccaaaggcccccgtgccactgctcccacccctgcccccacctccacctgagcccgagagctccgaggaccccaccagcccccctgagccccaggacttgagcagcagcgtctgcaaagaggagaagatgcccagaggaggctcactggagagcgacggctgccccaaggagccagctaagactcagcccgcggttgccaccgccgccacggccgcagaaaagtacaaacaccgaggggagggagagcgcaaagacattgtttcatcctccatgccaaggccaaacagagaggagcctgtggacagccggacgcccgtgaccgagagagttagcgggagctccggcagttctggagaacaaaaactcatctcagaagaggatctgtgaacaagaataaaggcagctgttgtctcttctccttatgggtagggctctgacaaagcttcccatatcaccaggactgttaatatatttaaaaacaaaaggcaatttattaaggaaatttgtaccagtgaattctaccagtgccatagtacctgtatacgtttcaaaaactcccttctttcctcccgtctacaccccccccccactgaatccaaacaccattgtcacactccacctgtaacctatttattaatgcccttttaacattgcactatataaagagtttgccttataaatttacataaaaatgtccgtttgtgtcttttgttg

SEQ ID NO: 56 - DNA, 2100 bp, synthetic construct
  source 1..2100: mol_type = other DNA
attgagggcgtcaccgctaaggctccgccccagcctgggctccacaaccaatgaagggtaatctcgacaaagagcaaggggtggggcgcgggcgcgcaggtgcagcagcacacaggctggtcgggagggcggggcgcgacgtctgccgtgcggggtcccggcatcggttgcgcgcgcgctccctcctctcggagagagggctgtggtaaaacccgtccggaaaccatggccgccgccgccgccgccgcgccgagcggaggaggaggaggaggcgaggaggagagactggaagaaaagtcagaagaccaggacctccagggcctcaaggacaaacccctcaagtttaaaaaggtgaagaaagataagaaagaagagaaagagggcaagcatgagcccgtgcagccatcagcccaccactctgctgagcccgcagaggcaggcaaagcagagacatcagaagggtcaggctccgccccggctgtgccggaagcttctgcctcccccaaacagcggcgctccatcatccgtgaccggggacccatgtatgatgaccccaccctgcctgaaggctggacacggaagcttaagcaaaggaaatctggccgctctgctgggaagtatgatgtgtatttgatcaatccccagggaaaagcctttcgctctaaagtggagttgattgcgtacttcgaaaaggtaggcgacacatccctggaccctaatgattttgacttcacggtaactgggagagggagcccctcccggcgagagcagaaaccacctaagaagcccaaatctcccaaagctccaggaactggcagaggccggggacgccccaaagggagcggcaccacgagacccaaggcggccacgtcagagggtgtgcaggtgaaaagggtcctggagaaaagtcctgggaagctccttgtcaagatgccttttcaaacttcgccagggggcaaggctgaggggggtggggccaccacatccacccaggtcatggtgatcaaacgccccggcaggaagcgaaaagctgaggccgaccctcaggccattcccaagaaacggggccgaaagccggggagtgtggtggcagccgctgccgccgaggccaaaaagaaagccgtgaaggagtcttctatccgatctgtgcaggagaccgtactccccatcaagaagcgcaagacccgggagacggtcagcatcgaggtcaaggaagtggtgaagcccctgctggtgtccaccctcggtgagaagagcgggaaaggactgaagacctgtaagagccctgggcggaaaagcaaggagagcagccccaaggggcgcagcagcagcgcctcctcaccccccaagaaggagcaccaccaccatcaccaccactcagagtccccaaaggcccccgtgccactgctcccacccctgcccccacctccacctgagcccgagagctccgaggaccccaccagcccccctgagccccaggacttgagcagcagcgtctgcaaagaggagaagatgcccagaggaggctcactggagagcgacggctgccccaaggagccagctaagactcagcccgcggttgccaccgccgccacggccgcagaaaagtacaaacaccgaggggagggagagcgcaaagacattgtttcatcctccatgccaaggccaaacagagaggagcctgtggacagccggacgcccgtgaccgagagagttagcgggagctccggcagttctggagaacaaaaactcatctcagaagaggatctgtgaacaagaataaaggcagctgttgtctcttctccttatgggtagggctctgacaaagcttcccatatcaccaggactgttaatatatttaaaaacaaaaggcaatttattaaggaaatttgtaccagtgaattctaccagtgccatagtacctgtatacgtttcaaaaactcccttctttcctcccgtctacaccccccccccactgaatccaaacaccattgtcacactccacctgtaacctatttattacgaccatggctgtagactgttatataaagagtttgccttataaatttacataaaaatgtccgtttgtgtcttttgttg

SEQ ID NO: 57 - DNA, 42 bp, synthetic construct
  source 1..42: mol_type = other DNA
caattcacgcgtgctagcataggcgccaagagcctagacttc

SEQ ID NO: 58 - DNA, 42 bp, synthetic construct
  source 1..42: mol_type = other DNA
caccatggtggcaagctttttccggacgggttttaccacagc

SEQ ID NO: 59 - DNA, 41 bp, synthetic construct
  source 1..41: mol_type = other DNA
catggacgagctgtacaaggggagctccggcagttctggag

SEQ ID NO: 60 - DNA, 49 bp, synthetic construct
  source 1..49: mol_type = other DNA
ttcctagtactgcggccgccacacaaaaaaccaacacacagatctaatg

SEQ ID NO: 61 - DNA, 53 bp, synthetic construct
  source 1..53: mol_type = other DNA
aactatacaacctactacctcagttttataaagagtttgccttataaatttac

SEQ ID NO: 62 - DNA, 49 bp, synthetic construct
  source 1..49: mol_type = other DNA
tgaggtagtaggttgtatagttccggttcagacaggtttactgaaatgg

SEQ ID NO: 63 - DNA, 53 bp, synthetic construct
  source 1..53: mol_type = other DNA
cacaagatcggatctacgggttgttttataaagagtttgccttataaatttac

SEQ ID NO: 64 - DNA, 49 bp, synthetic construct
  source 1..49: mol_type = other DNA
aacccgtagatccgatcttgtgccggttcagacaggtttactgaaatgg

SEQ ID NO: 65 - DNA, 53 bp, synthetic construct
  source 1..53: mol_type = other DNA
cacaagttcggatctacgggttgttttataaagagtttgccttataaatttac

SEQ ID NO: 66 - DNA, 49 bp, synthetic construct
  source 1..49: mol_type = other DNA
aacccgtagatccgaacttgtgccggttcagacaggtttactgaaatgg

SEQ ID NO: 67 - DNA, 54 bp, synthetic construct
  source 1..54: mol_type = other DNA
acaaggatgaatctttgttactggttttataaagagtttgccttataaatttac

SEQ ID NO: 68 - DNA, 50 bp, synthetic construct
  source 1..50: mol_type = other DNA
cagtaacaaagattcatccttgtccggttcagacaggtttactgaaatgg

SEQ ID NO: 69 - DNA, 53 bp, synthetic construct
  source 1..53: mol_type = other DNA
gaggctcagaatggctcaggaggttttataaagagtttgccttataaatttac

SEQ ID NO: 70 - DNA, 49 bp, synthetic construct
  source 1..49: mol_type = other DNA
ctcctgagccattctgagcctcccggttcagacaggtttactgaaatgg

SEQ ID NO: 71 - DNA, 4285 bp, synthetic construct
  source 1..4285: mol_type = other DNA
tcgcgcgtttcggtgatgacggtgaaaacctctgacacatgcagctcccggacgtcattgtcgatgctagcctgcgcgctcgctcgctcactgaggccgcccgggcaaagcccgggcgtcgggcgacctttggtcgcccggcctcagtgagcgagcgagcgcgcagagagggagtggataggcgccaagagcctagacttccttaagcgccagagtccacaagggcccagttaatcctcaacattcaaatgctgcccacaaaaccagcccctctgtgccctagccgcctcttttttccaagtgacagtagaactccaccaatccgcagctgaatggggtccgcctcttttccctgcctaaacagacaggaactcctgccaattgagggcgtcaccgctaaggctccgccccagcctgggctccacaaccaatgaagggtaatctcgacaaagagcaaggggtggggcgcgggcgcgcaggtgcagcagcacacaggctggtcgggagggcggggcgcgacgtctgccgtgcggggtcccggcatcggttgcgcgcgcgctccctcctctcggagagagggctgtggtaaaacccgtccggaaaccatggccgccgccgccgccgccgcgccgagcggaggaggaggaggaggcgaggaggagagactggaagaaaagtcagaagaccaggacctccagggcctcaaggacaaacccctcaagtttaaaaaggtgaagaaagataagaaagaagagaaagagggcaagcatgagcccgtgcagccatcagcccaccactctgctgagcccgcagaggcaggcaaagcagagacatcagaagggtcaggctccgccccggctgtgccggaagcttctgcctcccccaaacagcggcgctccatcatccgtgaccggggacccatgtatgatgaccccaccctgcctgaaggctggacacggaagcttaagcaaaggaaatctggccgctctgctgggaagtatgatgtgtatttgatcaatccccagggaaaagcctttcgctctaaagtggagttgattgcgtacttcgaaaaggtaggcgacacatccctggaccctaatgattttgacttcacggtaactgggagagggagcccctcccggcgagagcagaaaccacctaagaagcccaaatctcccaaagctccaggaactggcagaggccggggacgccccaaagggagcggcaccacgagacccaaggcggccacgtcagagggtgtgcaggtgaaaagggtcctggagaaaagtcctgggaagctccttgtcaagatgccttttcaaacttcgccagggggcaaggctgaggggggtggggccaccacatccacccaggtcatggtgatcaaacgccccggcaggaagcgaaaagctgaggccgaccctcaggccattcccaagaaacggggccgaaagccggggagtgtggtggcagccgctgccgccgaggccaaaaagaaagccgtgaaggagtcttctatccgatctgtgcaggagaccgtactccccatcaagaagcgcaagacccgggagacggtcagcatcgaggtcaaggaagtggtgaagcccctgctggtgtccaccctcggtgagaagagcgggaaaggactgaagacctgtaagagccctgggcggaaaagcaaggagagcagccccaaggggcgcagcagcagcgcctcctcaccccccaagaaggagcaccaccaccatcaccaccactcagagtccccaaaggcccccgtgccactgctcccacccctgcccccacctccacctgagcccgagagctccgaggaccccaccagcccccctgagccccaggacttgagcagcagcgtctgcaaagaggagaagatgcccagaggaggctcactggagagcgacggctgccccaaggagccagctaagactcagcccgcggttgccaccgccgccacggccgcagaaaagtacaaacaccgaggggagggagagcgcaaagacattgtttcatcctccatgccaaggccaaacagagaggagcctgtggacagccggacgcccgtgaccgagagagttagcgggagctccggcagttctggagaacaaaaactcatctcagaagaggatctgtgaacaagaataaaggcagctgttgtctcttctccttatgggtagggctctgacaaagcttcccatatcaccaggactgttaatatatttaaaaacaaaaggcaatttattaaggaaatttgtaccatttcagtaaacctgtctgaaccggaactatacaacctactacctcagttttataaagagtttgccttataaatttacataaaaatgtccgtttgtgtcttttgttgaggaacccctagtgatggagttggccactccctctctgcgcgctcgctcgctcactgaggccgggcgaccaaaggtcgcccgacgcccgggctttgcccgggcggcctcagtgagcgagcgagcgcgcagagagggagtggccatcattgtcacatgtgagcaaaaggccagcaaaaggccaggaaccgtaaaaaggccgcgttgctggcgtttttccataggctccgcccccctgacgagcatcacaaaaatcgacgctcaagtcagaggtggcgaaacccgacaggactataaagataccaggcgtttccccctggaagctccctcgtgcgctctcctgttccgaccctgccgcttaccggatacctgtccgcctttctcccttcgggaagcgtggcgctttctcatagctcacgctgtaggtatctcagttcggtgtaggtcgttcgctccaagctgggctgtgtgcacgaaccccccgttcagcccgaccgctgcgccttatccggtaactatcgtcttgagtccaacccggtaagacacgacttatcgccactggcagcagccactggtaacaggattagcagagcgaggtatgtaggcggtgctacagagttcttgaagtggtggcctaactacggctacactagaagaacagtatttggtatctgcgctctgctgaagccagttaccttcggaaaaagagttggtagctcttgatccggcaaacaaaccaccgctggtagcggtggtttttttgtttgcaagcagcagattacgcgcagaaaaaaaggatctcaagaagatcctttgatcttttctacggggtctgacgctcagtggaacgaaaactcacgttaagggattttggtcatgagattatcaaaaaggatcttcacctagatccttttaaattaaaaatgaagttttaaatcaagcccaatctgaataatgttacaaccaattaaccaattctgattagaaaaactcatcgagcatcaaatgaaactgcaatttattcatatcaggattatcaataccatatttttgaaaaagccgtttctgtaatgaaggagaaaactcaccgaggcagttccataggatggcaagatcctggtatcggtctgcgattccgactcgtccaacatcaatacaacctattaatttcccctcgtcaaaaataaggttatcaagtgagaaatcaccatgagtgacgactgaatccggtgagaatggcaaaagtttatgcatttctttccagacttgttcaacaggccagccattacgctcgtcatcaaaatcactcgcatcaaccaaaccgttattcattcgtgattgcgcctgagcgagacgaaatacgcgatcgctgttaaaaggacaattacaaacaggaatcgaatgcaaccggcgcaggaacactgccagcgcatcaacaatattttcacctgaatcaggatattcttctaatacctggaatgctgtttttccggggatcgcagtggtgagtaaccatgcatcatcaggagtacggataaaatgcttgatggtcggaagaggcataaattccgtcagccagtttagtctgaccatctcatctgtaacatcattggcaacgctacctttgccatgtttcagaaacaactctggcgcatcgggcttcccatacaagcgatagattgtcgcacctgattgcccgacattatcgcgagcccatttatacccatataaatcagcatccatgttggaatttaatcgcggcctcgacgtttcccgttgaatatggctcataacaccccttgtattactgtttatgtaagcagacagttttattgttcatgatgatatatttttatcttgtgcaatgtaacatcagagattttgagacacgggccagagctgca

SEQ ID NO: 72 - DNA, 4285 bp, synthetic construct
  source 1..4285: mol_type = other DNA
tcgcgcgtttcggtgatgacggtgaaaacctctgacacatgcagctcccggacgtcattgtcgatgctagcctgcgcgctcgctcgctcactgaggccgcccgggcaaagcccgggcgtcgggcgacctttggtcgcccggcctcagtgagcgagcgagcgcgcagagagggagtggataggcgccaagagcctagacttccttaagcgccagagtccacaagggcccagttaatcctcaacattcaaatgctgcccacaaaaccagcccctctgtgccctagccgcctcttttttccaagtgacagtagaactccaccaatccgcagctgaatggggtccgcctcttttccctgcctaaacagacaggaactcctgccaattgagggcgtcaccgctaaggctccgccccagcctgggctccacaaccaatgaagggtaatctcgacaaagagcaaggggtggggcgcgggcgcgcaggtgcagcagcacacaggctggtcgggagggcggggcgcgacgtctgccgtgcggggtcccggcatcggttgcgcgcgcgctccctcctctcggagagagggctgtggtaaaacccgtccggaaaccatggccgccgccgccgccgccgcgccgagcggaggaggaggaggaggcgaggaggagagactggaagaaaagtcagaagaccaggacctccagggcctcaaggacaaacccctcaagtttaaaaaggtgaagaaagataagaaagaagagaaagagggcaagcatgagcccgtgcagccatcagcccaccactctgctgagcccgcagaggcaggcaaagcagagacatcagaagggtcaggctccgccccggctgtgccggaagcttctgcctcccccaaacagcggcgctccatcatccgtgaccggggacccatgtatgatgaccccaccctgcctgaaggctggacacggaagcttaagcaaaggaaatctggccgctctgctgggaagtatgatgtgtatttgatcaatccccagggaaaagcctttcgctctaaagtggagttgattgcgtacttcgaaaaggtaggcgacacatccctggaccctaatgattttgacttcacggtaactgggagagggagcccctcccggcgagagcagaaaccacctaagaagcccaaatctcccaaagctccaggaactggcagaggccggggacgccccaaagggagcggcaccacgagacccaaggcggccacgtcagagggtgtgcaggtgaaaagggtcctggagaaaagtcctgggaagctccttgtcaagatgccttttcaaacttcgccagggggcaaggctgaggggggtggggccaccacatccacccaggtcatggtgatcaaacgccccggcaggaagcgaaaagctgaggccgaccctcaggccattcccaagaaacggggccgaaagccggggagtgtggtggcagccgctgccgccgaggccaaaaagaaagccgtgaaggagtcttctatccgatctgtgcaggagaccgtactccccatcaagaagcgcaagacccgggagacggtcagcatcgaggtcaaggaagtggtgaagcccctgctggtgtccaccctcggtgagaagagcgggaaaggactgaagacctgtaagagccctgggcggaaaagcaaggagagcagccccaaggggcgcagcagcagcgcctcctcaccccccaagaaggagcaccaccaccatcaccaccactcagagtccccaaaggcccccgtgccactgctcccacccctgcccccacctccacctgagcccgagagctccgaggaccccaccagcccccctgagccccaggacttgagcagcagcgtctgcaaagaggagaagatgcccagaggaggctcactggagagcgacggctgccccaaggagccagctaagactcagcccgcggttgccaccgccgccacggccgcagaaaagtacaaacaccgaggggagggagagcgcaaagacattgtttcatcctccatgccaaggccaaacagagaggagcctgtggacagccggacgcccgtgaccgagagagttagcgggagctccggcagttctggagaacaaaaactcatctcagaagaggatctgtgaacaagaataaaggcagctgttgtctcttctccttatgggtagggctctgacaaagcttcccatatcaccaggactgttaatatatttaaaaacaaaaggcaatttattaaggaaatttgtaccatttcagtaaacctgtctgaaccggcacaagatcggatctacgggttgttttataaagagtttgccttataaatttacataaaaatgtccgtttgtgtcttttgttgaggaacccctagtgatggagttggccactccctctctgcgcgctcgctcgctcactgaggccgggcgaccaaaggtcgcccgacgcccgggctttgcccgggcggcctcagtgagcgagcgagcgcgcagagagggagtggccatcattgtcacatgtgagcaaaaggccagcaaaaggccaggaaccgtaaaaaggccgcgttgctggcgtttttccataggctccgcccccctgacgagcatcacaaaaatcgacgctcaagtcagaggtggcgaaacccgacaggactataaagataccaggcgtttccccctggaagctccctcgtgcgctctcctgttccgaccctgccgcttaccggatacctgtccgcctttctcccttcgggaagcgtggcgctttctcatagctcacgctgtaggtatctcagttcggtgtaggtcgttcgctccaagctgggctgtgtgcacgaaccccccgttcagcccgaccgctgcgccttatccggtaactatcgtcttgagtccaacccggtaagacacgacttatcgccactggcagcagccactggtaacaggattagcagagcgaggtatgtaggcggtgctacagagttcttgaagtggtggcctaactacggctacactagaagaacagtatttggtatctgcgctctgctgaagccagttaccttcggaaaaagagttggtagctcttgatccggcaaacaaaccaccgctggtagcggtggtttttttgtttgcaagcagcagattacgcgcagaaaaaaaggatctcaagaagatcctttgatcttttctacggggtctgacgctcagtggaacgaaaactcacgttaagggattttggtcatgagattatcaaaaaggatcttcacctagatccttttaaattaaaaatgaagttttaaatcaagcccaatctgaataatgttacaaccaattaaccaattctgattagaaaaactcatcgagcatcaaatgaaactgcaatttattcatatcaggattatcaataccatatttttgaaaaagccgtttctgtaatgaaggagaaaactcaccgaggcagttccataggatggcaagatcctggtatcggtctgcgattccgactcgtccaacatcaatacaacctattaatttcccctcgtcaaaaataaggttatcaagtgagaaatcaccatgagtgacgactgaatccggtgagaatggcaaaagtttatgcatttctttccagacttgttcaacaggccagccattacgctcgtcatcaaaatcactcgcatcaaccaaaccgttattcattcgtgattgcgcctgagcgagacgaaatacgcgatcgctgttaaaaggacaattacaaacaggaatcgaatgcaaccggcgcaggaacactgccagcgcatcaacaatattttcacctgaatcaggatattcttctaatacctggaatgctgtttttccggggatcgcagtggtgagtaaccatgcatcatcaggagtacggataaaatgcttgatggtcggaagaggcataaattccgtcagccagtttagtctgaccatctcatctgtaacatcattggcaacgctacctttgccatgtttcagaaacaactctggcgcatcgggcttcccatacaagcgatagattgtcgcacctgattgcccgacattatcgcgagcccatttatacccatataaatcagcatccatgttggaatttaatcgcggcctcgacgtttcccgttgaatatggctcataacaccccttgtattactgtttatgtaagcagacagttttattgttcatgatgatatatttttatcttgtgcaatgtaacatcagagattttgagacacgggccagagctgca

SEQ ID NO: 73 - DNA, 4285 bp, synthetic construct
  source 1..4285: mol_type = other DNA
tcgcgcgtttcggtgatgacggtgaaaacctctgacacatgcagctcccggacgtcattgtcgatgctagcctgcgcgctcgctcgctcactgaggccgcccgggcaaagcccgggcgtcgggcgacctttggtcgcccggcctcagtgagcgagcgagcgcgcagagagggagtggataggcgccaagagcctagacttccttaagcgccagagtccacaagggcccagttaatcctcaacattcaaatgctgcccacaaaaccagcccctctgtgccctagccgcctcttttttccaagtgacagtagaactccaccaatccgcagctgaatggggtccgcctcttttccctgcctaaacagacaggaactcctgccaattgagggcgtcaccgctaaggctccgccccagcctgggctccacaaccaatgaagggtaatctcgacaaagagcaaggggtggggcgcgggcgcgcaggtgcagcagcacacaggctggtcgggagggcggggcgcgacgtctgccgtgcggggtcccggcatcggttgcgcgcgcgctccctcctctcggagagagggctgtggtaaaacccgtccggaaaccatggccgccgccgccgccgccgcgccgagcggaggaggaggaggaggcgaggaggagagactggaagaaaagtcagaagaccaggacctccagggcctcaaggacaaacccctcaagtttaaaaaggtgaagaaagataagaaagaagagaaagagggcaagcatgagcccgtgcagccatcagcccaccactctgctgagcccgcagaggcaggcaaagcagagacatcagaagggtcaggctccgccccggctgtgccggaagcttctgcctcccccaaacagcggcgctccatcatccgtgaccggggacccatgtatgatgaccccaccctgcctgaaggctggacacggaagcttaagcaaaggaaatctggccgctctgctgggaagtatgatgtgtatttgatcaatccccagggaaaagcctttcgctctaaagtggagttgattgcgtacttcgaaaaggtaggcgacacatccctggaccctaatgattttgacttcacggtaactgggagagggagcccctcccggcgagagcagaaaccacctaagaagcccaaatctcccaaagctccaggaactggcagaggccggggacgccccaaagggagcggcaccacgagacccaaggcggccacgtcagagggtgtgcaggtgaaaagggtcctggagaaaagtcctgggaagctccttgtcaagatgccttttcaaacttcgccagggggcaaggctgaggggggtggggccaccacatccacccaggtcatggtgatcaaacgccccggcaggaagcgaaaagctgaggccgaccctcaggccattcccaagaaacggggccgaaagccggggagtgtggtggcagccgctgccgccgaggccaaaaagaaagccgtgaaggagtcttctatccgatctgtgcaggagaccgtactccccatcaagaagcgcaagacccgggagacggtcagcatcgaggtcaaggaagtggtgaagcccctgctggtgtccaccctcggtgagaagagcgggaaaggactgaagacctgtaagagccctgggcggaaaagcaaggagagcagccccaaggggcgcagcagcagcgcctcctcaccccccaagaaggagcaccaccaccatcaccaccactcagagtccccaaaggcccccgtgccactgctcccacccctgcccccacctccacctgagcccgagagctccgaggaccccaccagcccccctgagccccaggacttgagcagcagcgtctgcaaagaggagaagatgcccagaggaggctcactggagagcgacggctgccccaaggagccagctaagactcagcccgcggttgccaccgccgccacggccgcagaaaagtacaaacaccgaggggagggagagcgcaaagacattgtttcatcctccatgccaaggccaaacagagaggagcctgtggacagccggacgcccgtgaccgagagagttagcgggagctccggcagttctggagaacaaaaactcatctcagaagaggatctgtgaacaagaataaaggcagctgttgtctcttctccttatgggtagggctctgacaaagcttcccatatcaccaggactgttaatatatttaaaaacaaaaggcaatttattaaggaaatttgtaccatttcagtaaacctgtctgaaccggcacaagttcggatctacgggttgttttataaagagtttgccttataaatttacataaaaatgtccgtttgtgtcttttgttgaggaacccctagtgatggagttggccactccctctctgcgcgctcgctcgctcactgaggccgggcgaccaaaggtcgcccgacgcccgggctttgcccgggcggcctcagtgagcgagcgagcgcgcagagagggagtggccatcattgtcacatgtgagcaaaaggccagcaaaaggccaggaaccgtaaaaaggccgcgttgctggcgtttttccataggctccgcccccctgacgagcatcacaaaaatcgacgctcaagtcagaggtggcgaaacccgacaggactataaagataccaggcgtttccccctggaagctccctcgtgcgctctcctgttccgaccctgccgcttaccggatacctgtccgcctttctcccttcgggaagcgtggcgctttctcatagctcacgctgtaggtatctcagttcggtgtaggtcgttcgctccaagctgggctgtgtgcacgaaccccccgttcagcccgaccgctgcgccttatccggtaactatcgtcttgagtccaacccggtaagacacgacttatcgccactggcagcagccactggtaacaggattagcagagcgaggtatgtaggcggtgctacagagttcttgaagtggtggcctaactacggctacactagaagaacagtatttggtatctgcgctctgctgaagccagttaccttcggaaaaagagttggtagctcttgatccggcaaacaaaccaccgctggtagcggtggtttttttgtttgcaagcagcagattacgcgcagaaaaaaaggatctcaagaagatcctttgatcttttctacggggtctgacgctcagtggaacgaaaactcacgttaagggattttggtcatgagattatcaaaaaggatcttcacctagatccttttaaattaaaaatgaagttttaaatcaagcccaatctgaataatgttacaaccaattaaccaattctgattagaaaaactcatcgagcatcaaatgaaactgcaatttattcatatcaggattatcaataccatatttttgaaaaagccgtttctgtaatgaaggagaaaactcaccgaggcagttccataggatggcaagatcctggtatcggtctgcgattccgactcgtccaacatcaatacaacctattaatttcccctcgtcaaaaataaggttatcaagtgagaaatcaccatgagtgacgactgaatccggtgagaatggcaaaagtttatgcatttctttccagacttgttcaacaggccagccattacgctcgtcatcaaaatcactcgcatcaaccaaaccgttattcattcgtgattgcgcctgagcgagacgaaatacgcgatcgctgttaaaaggacaattacaaacaggaatcgaatgcaaccggcgcaggaacactgccagcgcatcaacaatattttcacctgaatcaggatattcttctaatacctggaatgctgtttttccggggatcgcagtggtgagtaaccatgcatcatcaggagtacggataaaatgcttgatggtcggaagaggcataaattccgtcagccagtttagtctgaccatctcatctgtaacatcattggcaacgctacctttgccatgtttcagaaacaactctggcgcatcgggcttcccatacaagcgatagattgtcgcacctgattgcccgacattatcgcgagcccatttatacccatataaatcagcatccatgttggaatttaatcgcggcctcgacgtttcccgttgaatatggctcataacaccccttgtattactgtttatgtaagcagacagttttattgttcatgatgatatatttttatcttgtgcaatgtaacatcagagattttgagacacgggccagagctgca

SEQ ID NO: 74 - DNA, 4286 bp, synthetic construct
  source 1..4286: mol_type = other DNA
tcgcgcgtttcggtgatgacggtgaaaacctctgacacatgcagctcccggacgtcattgtcgatgctagcctgcgcgctcgctcgctcactgaggccgcccgggcaaagcccgggcgtcgggcgacctttggtcgcccggcctcagtgagcgagcgagcgcgcagagagggagtggataggcgccaagagcctagacttccttaagcgccagagtccacaagggcccagttaatcctcaacattcaaatgctgcccacaaaaccagcccctctgtgccctagccgcctcttttttccaagtgacagtagaactccaccaatccgcagctgaatggggtccgcctcttttccctgcctaaacagacaggaactcctgccaattgagggcgtcaccgctaaggctccgccccagcctgggctccacaaccaatgaagggtaatctcgacaaagagcaaggggtggggcgcgggcgcgcaggtgcagcagcacacaggctggtcgggagggcggggcgcgacgtctgccgtgcggggtcccggcatcggttgcgcgcgcgctccctcctctcggagagagggctgtggtaaaacccgtccggaaaccatggccgccgccgccgccgccgcgccgagcggaggaggaggaggaggcgaggaggagagactggaagaaaagtcagaagaccaggacctccagggcctcaaggacaaacccctcaagtttaaaaaggtgaagaaagataagaaagaagagaaagagggcaagcatgagcccgtgcagccatcagcccaccactctgctgagcccgcagaggcaggcaaagcagagacatcagaagggtcaggctccgccccggctgtgccggaagcttctgcctcccccaaacagcggcgctccatcatccgtgaccggggacccatgtatgatgaccccaccctgcctgaaggctggacacggaagcttaagcaaaggaaatctggccgctctgctgggaagtatgatgtgtatttgatcaatccccagggaaaagcctttcgctctaaagtggagttgattgcgtacttcgaaaaggtaggcgacacatccctggaccctaatgattttgacttcacggtaactgggagagggagcccctcccggcgagagcagaaaccacctaagaagcccaaatctcccaaagctccaggaactggcagaggccggggacgccccaaagggagcggcaccacgagacccaaggcggccacgtcagagggtgtgcaggtgaaaagggtcctggagaaaagtcctgggaagctccttgtcaagatgccttttcaaacttcgccagggggcaaggctgaggggggtggggccaccacatccacccaggtcatggtgatcaaacgccccggcaggaagcgaaaagctgaggccgaccctcaggccattcccaagaaacggggccgaaagccggggagtgtggtggcagccgctgccgccgaggccaaaaagaaagccgtgaaggagtcttctatccgatctgtgcaggagaccgtactccccatcaagaagcgcaagacccgggagacggtcagcatcgaggtcaaggaagtggtgaagcccctgctggtgtccaccctcggtgagaagagcgggaaaggactgaagacctgtaagagccctgggcggaaaagcaaggagagcagccccaaggggcgcagcagcagcgcctcctcaccccccaagaaggagcaccaccaccatcaccaccactcagagtccccaaaggcccccgtgccactgctcccacccctgcccccacctccacctgagcccgagagctccgaggaccccaccagcccccctgagccccaggacttgagcagcagcgtctgcaaagaggagaagatgcccagaggaggctcactggagagcgacggctgccccaaggagccagctaagactcagcccgcggttgccaccgccgccacggccgcagaaaagtacaaacaccgaggggagggagagcgcaaagacattgtttcatcctccatgccaaggccaaacagagaggagcctgtggacagccggacgcccgtgaccgagagagttagcgggagctccggcagttctggagaacaaaaactcatctcagaagaggatctgtgaacaagaataaaggcagctgttgtctcttctccttatgggtagggctctgacaaagcttcccatatcaccaggactgttaatatatttaaaaacaaaaggcaatttattaaggaaatttgtaccatttcagtaaacctgtctgaaccggacaaggatgaatctttgttactggttttataaagagtttgccttataaatttacataaaaatgtccgtttgtgtcttttgttgaggaacccctagtgatggagttggccactccctctctgcgcgctcgctcgctcactgaggccgggcgaccaaaggtcgcccgacgcccgggctttgcccgggcggcctcagtgagcgagcgagcgcgcagagagggagtggccatcattgtcacatgtgagcaaaaggccagcaaaaggccaggaaccgtaaaaaggccgcgttgctggcgtttttccataggctccgcccccctgacgagcatcacaaaaatcgacgctcaagtcagaggtggcgaaacccgacaggactataaagataccaggcgtttccccctggaagctccctcgtgcgctctcctgttccgaccctgccgcttaccggatacctgtccgcctttctcccttcgggaagcgtggcgctttctcatagctcacgctgtaggtatctcagttcggtgtaggtcgttcgctccaagctgggctgtgtgcacgaaccccccgttcagcccgaccgctgcgccttatccggtaactatcgtcttgagtccaacccggtaagacacgacttatcgccactggcagcagccactggtaacaggattagcagagcgaggtatgtaggcggtgctacagagttcttgaagtggtggcctaactacggctacactagaagaacagtatttggtatctgcgctctgctgaagccagttaccttcggaaaaagagttggtagctcttgatccggcaaacaaaccaccgctggtagcggtggtttttttgtttgcaagcagcagattacgcgcagaaaaaaaggatctcaagaagatcctttgatcttttctacggggtctgacgctcagtggaacgaaaactcacgttaagggattttggtcatgagattatcaaaaaggatcttcacctagatccttttaaattaaaaatgaagttttaaatcaagcccaatctgaataatgttacaaccaattaaccaattctgattagaaaaactcatcgagcatcaaatgaaactgcaatttattcatatcaggattatcaataccatatttttgaaaaagccgtttctgtaatgaaggagaaaactcaccgaggcagttccataggatggcaagatcctggtatcggtctgcgattccgactcgtccaacatcaatacaacctattaatttcccctcgtcaaaaataaggttatcaagtgagaaatcaccatgagtgacgactgaatccggtgagaatggcaaaagtttatgcatttctttccagacttgttcaacaggccagccattacgctcgtcatcaaaatcactcgcatcaaccaaaccgttattcattcgtgattgcgcctgagcgagacgaaatacgcgatcgctgttaaaaggacaattacaaacaggaatcgaatgcaaccggcgcaggaacactgccagcgcatcaacaatattttcacctgaatcaggatattcttctaatacctggaatgctgtttttccggggatcgcagtggtgagtaaccatgcatcatcaggagtacggataaaatgcttgatggtcggaagaggcataaattccgtcagccagtttagtctgaccatctcatctgtaacatcattggcaacgctacctttgccatgtttcagaaacaactctggcgcatcgggcttcccatacaagcgatagattgtcgcacctgattgcccgacattatcgcgagcccatttatacccatataaatcagcatccatgttggaatttaatcgcggcctcgacgtttcccgttgaatatggctcataacaccccttgtattactgtttatgtaagcagacagttttattgttcatgatgatatatttttatcttgtgcaatgtaacatcagagattttgagacacgggccagagctgca

SEQ ID NO: 75 - DNA, 4285 bp, synthetic construct
  source 1..4285: mol_type = other DNA
tcgcgcgtttcggtgatgacggtgaaaacctctgacacatgcagctcccggacgtcattgtcgatgctagcctgcgcgctcgctcgctcactgaggccgcccgggcaaagcccgggcgtcgggcgacctttggtcgcccggcctcagtgagcgagcgagcgcgcagagagggagtggataggcgccaagagcctagacttccttaagcgccagagtccacaagggcccagttaatcctcaacattcaaatgctgcccacaaaaccagcccctctgtgccctagccgcctcttttttccaagtgacagtagaactccaccaatccgcagctgaatggggtccgcctcttttccctgcctaaacagacaggaactcctgccaattgagggcgtcaccgctaaggctccgccccagcctgggctccacaaccaatgaagggtaatctcgacaaagagcaaggggtggggcgcgggcgcgcaggtgcagcagcacacaggctggtcgggagggcggggcgcgacgtctgccgtgcggggtcccggcatcggttgcgcgcgcgctccctcctctcggagagagggctgtggtaaaacccgtccggaaaccatggccgccgccgccgccgccgcgccgagcggaggaggaggaggaggcgaggaggagagactggaagaaaagtcagaagaccaggacctccagggcctcaaggacaaacccctcaagtttaaaaaggtgaagaaagataagaaagaagagaaagagggcaagcatgagcccgtgcagccatcagcccaccactctgctgagcccgcagaggcaggcaaagcagagacatcagaagggtcaggctccgccccggctgtgccggaagcttctgcctcccccaaacagcggcgctccatcatccgtgaccggggacccatgtatgatgaccccaccctgcctgaaggctggacacggaagcttaagcaaaggaaatctggccgctctgctgggaagtatgatgtgtatttgatcaatccccagggaaaagcctttcgctctaaagtggagttgattgcgtacttcgaaaaggtaggcgacacatccctggaccctaatgattttgacttcacggtaactgggagagggagcccctcccggcgagagcagaaaccacctaagaagcccaaatctcccaaagctccaggaactggcagaggccggggacgccccaaagggagcggcaccacgagacccaaggcggccacgtcagagggtgtgcaggtgaaaagggtcctggagaaaagtcctgggaagctccttgtcaagatgccttttcaaacttcgccagggggcaaggctgaggggggtggggccaccacatccacccaggtcatggtgatcaaacgccccggcaggaagcgaaaagctgaggccgaccctcaggccattcccaagaaacggggccgaaagccggggagtgtggtggcagccgctgccgccgaggccaaaaagaaagccgtgaaggagtcttctatccgatctgtgcaggagaccgtactccccatcaagaagcgcaagacccgggagacggtcagcatcgaggtcaaggaagtggtgaagcccctgctggtgtccaccctcggtgagaagagcgggaaaggactgaagacctgtaagagccctgggcggaaaagcaaggagagcagccccaaggggcgcagcagcagcgcctcctcaccccccaagaaggagcaccaccaccatcaccaccactcagagtccccaaaggcccccgtgccactgctcccacccctgcccccacctccacctgagcccgagagctccgaggaccccaccagcccccctgagccccaggacttgagcagcagcgtctgcaaagaggagaagatgcccagaggaggctcactggagagcgacggctgccccaaggagccagctaagactcagcccgcggttgccaccgccgccacggccgcagaaaagtacaaacaccgaggggagggagagcgcaaagacattgtttcatcctccatgccaaggccaaacagagaggagcctgtggacagccggacgcccgtgaccgagagagttagcgggagctccggcagttctggagaacaaaaactcatctcagaagaggatctgtgaacaagaataaaggcagctgttgtctcttctccttatgggtagggctctgacaaagcttcccatatcaccaggactgttaatatatttaaaaacaaaaggcaatttattaaggaaatttgtaccatttcagtaaacctgtctgaaccgggaggctcagaatggctcaggaggttttataaagagtttgccttataaatttacataaaaatgtccgtttgtgtcttttgttgaggaacccctagtgatggagttggccactccctctctgcgcgctcgctcgctcactgaggccgggcgaccaaaggtcgcccgacgcccgggctttgcccgggcggcctcagtgagcgagcgagcgcgcagagagggagtggccatcattgtcacatgtgagcaaaaggccagcaaaaggccaggaaccgtaaaaaggccgcgttgctggcgtttttccataggctccgcccccctgacgagcatcacaaaaatcgacgctcaagtcagaggtggcgaaacccgacaggactataaagataccaggcgtttccccctggaagctccctcgtgcgctctcctgttccgaccctgccgcttaccggatacctgtccgcctttctcccttcgggaagcgtggcgctttctcatagctcacgctgtaggtatctcagttcggtgtaggtcgttcgctccaagctgggctgtgtgcacgaaccccccgttcagcccgaccgctgcgccttatccggtaactatcgtcttgagtccaacccggtaagacacgacttatcgccactggcagcagccactggtaacaggattagcagagcgaggtatgtaggcggtgctacagagttcttgaagtggtggcctaactacggctacactagaagaacagtatttggtatctgcgctctgctgaagccagttaccttcggaaaaagagttggtagctcttgatccggcaaacaaaccaccgctggtagcggtggtttttttgtttgcaagcagcagattacgcgcagaaaaaaaggatctcaagaagatcctttgatcttttctacggggtctgacgctcagtggaacgaaaactcacgttaagggattttggtcatgagattatcaaaaaggatcttcacctagatccttttaaattaaaaatgaagttttaaatcaagcccaatctgaataatgttacaaccaattaaccaattctgattagaaaaactcatcgagcatcaaatgaaactgcaatttattcatatcaggattatcaataccatatttttgaaaaagccgtttctgtaatgaaggagaaaactcaccgaggcagttccataggatggcaagatcctggtatcggtctgcgattccgactcgtccaacatcaatacaacctattaatttcccctcgtcaaaaataaggttatcaagtgagaaatcaccatgagtgacgactgaatccggtgagaatggcaaaagtttatgcatttctttccagacttgttcaacaggccagccattacgctcgtcatcaaaatcactcgcatcaaccaaaccgttattcattcgtgattgcgcctgagcgagacgaaatacgcgatcgctgttaaaaggacaattacaaacaggaatcgaatgcaaccggcgcaggaacactgccagcgcatcaacaatattttcacctgaatcaggatattcttctaatacctggaatgctgtttttccggggatcgcagtggtgagtaaccatgcatcatcaggagtacggataaaatgcttgatggtcggaagaggcataaattccgtcagccagtttagtctgaccatctcatctgtaacatcattggcaacgctacctttgccatgtttcagaaacaactctggcgcatcgggcttcccatacaagcgatagattgtcgcacctgattgcccgacattatcgcgagcccatttatacccatataaatcagcatccatgttggaatttaatcgcggcctcgacgtttcccgttgaatatggctcataacaccccttgtattactgtttatgtaagcagacagttttattgttcatgatgatatatttttatcttgtgcaatgtaacatcagagattttgagacacgggccagagctgca